European Patent Specification EP 3 502 261 B1, published January 15, 2025. Title: Engineered Neovascularization-controling system. Applicant: Toolgen Inc. The sequence listing filed with the application follows.

SEQUENCE LISTING (1522 sequences)

SEQ ID NO: 1 - DNA, 22 bp, homo sapiens
gtagagcagcaaggcaaggctc

SEQ ID NO: 2 - DNA, 22 bp, homo sapiens
ctttctgtcctcagtggtccca

SEQ ID NO: 3 - DNA, 22 bp, homo sapiens
gagaccctggtggacatcttcc

SEQ ID NO: 4 - DNA, 22 bp, homo sapiens
ttccaggagtaccctgatgaga

SEQ ID NO: 5 - DNA, 22 bp, homo sapiens
ttgaagatgtactcgatctcat

SEQ ID NO: 6 - DNA, 22 bp, homo sapiens
aggggcacacaggatggcttga

SEQ ID NO: 7 - DNA, 22 bp, homo sapiens
agcagcccccgcatcgcatcag

SEQ ID NO: 8 - DNA, 22 bp, homo sapiens
gcagcagcccccgcatcgcatc

SEQ ID NO: 9 - DNA, 22 bp, homo sapiens
gtgatgttggactcctcagtgg

SEQ ID NO: 10 - DNA, 22 bp, homo sapiens
tggtgatgttggactcctcagt

SEQ ID NO: 11 - DNA, 22 bp, homo sapiens
catggtgatgttggactcctca

SEQ ID NO: 12 - DNA, 22 bp, homo sapiens
atgcggatcaaacctcaccaag

SEQ ID NO: 13 - DNA, 22 bp, homo sapiens
cacataggagagatgagcttcc

SEQ ID NO: 14 - DNA, 22 bp, homo sapiens
actcaccagcatccagaagttt

SEQ ID NO: 15 - DNA, 22 bp, homo sapiens
atttggatattgaagatgacat

SEQ ID NO: 16 - DNA, 22 bp, homo sapiens
atttacatttctgataatgtga

SEQ ID NO: 17 - DNA, 22 bp, homo sapiens
atgtgtttacagtttgaactaa

SEQ ID NO: 18 - DNA, 22 bp, homo sapiens
ctgtgtccagttagttcaaact

SEQ ID NO: 19 - DNA, 22 bp, homo sapiens
atggtcacatggatgagtaaaa

SEQ ID NO: 20 - DNA, 22 bp, homo sapiens
catgaggaaatgagagaaatgc

SEQ ID NO: 21 - DNA, 22 bp, homo sapiens
cccagtgagaaaagggaaagaa

SEQ ID NO: 22 - DNA, 22 bp, homo sapiens
ttgtgaaaaagggtaaagaaca

SEQ ID NO: 23 - DNA, 22 bp, homo sapiens
atagttcttcctcggctagtta

SEQ ID NO: 24 - DNA, 22 bp, homo sapiens
tcatagttcttcctcggctagt

SEQ ID NO: 25 - DNA, 22 bp, homo sapiens
tgttcttcatacacaggtattg

SEQ ID NO: 26 - DNA, 22 bp, homo sapiens
tacgtgaatgtggcctgtgcag

SEQ ID NO: 27 - DNA, 22 bp, homo sapiens
ctgcacaggccacattcacgta

SEQ ID NO: 28 - DNA, 22 bp, homo sapiens
ctgaggttggttactgttggta

SEQ ID NO: 29 - DNA, 22 bp, homo sapiens
caggtcataggtggtttcttat

SEQ ID NO: 30 - DNA, 22 bp, homo sapiens
accaagcaggtcataggtggtt

SEQ ID NO: 31 - DNA, 22 bp, homo sapiens
ttagatagcaagactttcctca

SEQ ID NO: 32 - DNA, 22 bp, homo sapiens
tcaggtccagcatgggtcctgc

SEQ ID NO: 33 - DNA, 22 bp, homo sapiens
cggcgcgtccctctgcacagca

SEQ ID NO: 34 - DNA, 22 bp, homo sapiens
gctgtgcagagggacgcgccgc

SEQ ID NO: 35 - DNA, 22 bp, homo sapiens
atcgtattcgagcggcgcgtcc

SEQ ID NO: 36 - DNA, 22 bp, homo sapiens
gatgttctccagcacttgcagc

SEQ ID NO: 37 - DNA, 22 bp, homo sapiens
agtgctggagaacatcatggaa

SEQ ID NO: 38 - DNA, 22 bp, homo sapiens
acaacatgaagaaagaaatggt

SEQ ID NO: 39 - DNA, 22 bp, homo sapiens
aaatggtagagatacagcagaa

SEQ ID NO: 40 - DNA, 22 bp, homo sapiens
ttctatcatcacagccgtctgg

SEQ ID NO: 41 - DNA, 22 bp, homo sapiens
aagttcaagtctcgtggtctga

SEQ ID NO: 42 - DNA, 22 bp, homo sapiens
acgagacttgaacttcagctct

SEQ ID NO: 43 - DNA, 22 bp, homo sapiens
aagaaggtgctagctatggaag

SEQ ID NO: 44 - DNA, 22 bp, homo sapiens
gatgatgtgcttgtcttccata

SEQ ID NO: 45 - DNA, 22 bp, homo sapiens
aacacctccgtctccttgctcc

SEQ ID NO: 46 - DNA, 22 bp, homo sapiens
gaagctgaccagcagatggaca

SEQ ID NO: 47 - DNA, 22 bp, homo sapiens
gcaatgaaaccctccaaggctt

SEQ ID NO: 48 - DNA, 22 bp, homo sapiens
aaaacatcagcaagttcatggg

SEQ ID NO: 49 - DNA, 22 bp, homo sapiens
gcaagttcatgggacttacaca

SEQ ID NO: 50 - DNA, 22 bp, homo sapiens
ggtcgcagggatgagtgaagtc

SEQ ID NO: 51 - DNA, 22 bp, homo sapiens
gcgggacttcttcatgaggatg

SEQ ID NO: 52 - DNA, 22 bp, homo sapiens
gaagtgcacggtcaccaacaga

SEQ ID NO: 53 - DNA, 22 bp, homo sapiens
acagtacggcctctgttggtga

SEQ ID NO: 54 - DNA, 22 bp, homo sapiens
tccaggtggctgacttgaggtt

SEQ ID NO: 55 - DNA, 22 bp, homo sapiens
caggacagcaggggctccttgt

SEQ ID NO: 56 - DNA, 22 bp, homo sapiens
tagcccccatgctttgcgagca

SEQ ID NO: 57 - DNA, 22 bp, homo sapiens
gcatcagggctgccccggccgt

SEQ ID NO: 58 - DNA, 22 bp, homo sapiens
gcatcagggctgccccggccgt

SEQ ID NO: 59 - DNA, 22 bp, homo sapiens
ggacgcaaagcgcggcgacttg

SEQ ID NO: 60 - DNA, 22 bp, homo sapiens
tcctgggacgagatgaatgtcc

SEQ ID NO: 61 - DNA, 22 bp, homo sapiens
ctgcagctcggccaggggctgc

SEQ ID NO: 62 - DNA, 22 bp, homo sapiens
ccaggggctgcgcgaacacgcg

SEQ ID NO: 63 - DNA, 22 bp, homo sapiens
ccctcggttccctgacaggcgg

SEQ ID NO: 64 - DNA, 22 bp, homo sapiens
accctgaggtccttcacagcct

SEQ ID NO: 65 - DNA, 22 bp, homo sapiens
ttccacaaggtggcccagcagc

SEQ ID NO: 66 - DNA, 22 bp, homo sapiens
cagcagcagcggcacctggaga

SEQ ID NO: 67 - DNA, 22 bp, homo sapiens
tcctagtttggcctcctggacc

SEQ ID NO: 68 - DNA, 22 bp, homo sapiens
gacccggctcacaatgtcagcc

SEQ ID NO: 69 - DNA, 22 bp, homo sapiens
gctgttgcggtcccccgtgatg

SEQ ID NO: 70 - DNA, 22 bp, homo sapiens
ggcgttgccatcccagtcccgc

SEQ ID NO: 71 - DNA, 22 bp, homo sapiens
aacgccgagttgctgcagttct

SEQ ID NO: 72 - DNA, 22 bp, homo sapiens
ataggccgtgtcctcgccaccc

SEQ ID NO: 73 - DNA, 22 bp, homo sapiens
gttctccgtgcacctgggtggc

SEQ ID NO: 74 - DNA, 22 bp, homo sapiens
acacggcctatagcctgcagct

SEQ ID NO: 75 - DNA, 22 bp, homo sapiens
ccaccgtcccacccagcggcct

SEQ ID NO: 76 - DNA, 22 bp, homo sapiens
gtgatcctggtcccaagtggag

SEQ ID NO: 77 - DNA, 22 bp, homo sapiens
gaccccggcaggaggctggtgg

SEQ ID NO: 78 - DNA, 22 bp, homo sapiens
tgcagccattccaacctcaacg

SEQ ID NO: 79 - DNA, 22 bp, homo sapiens
tgccgctgctgtgggatggagc

SEQ ID NO: 80 - DNA, 22 bp, homo sapiens
aaatcccggtataagtcctgga

SEQ ID NO: 81 - DNA, 22 bp, homo sapiens
gcaccaacgtacacgctccagg

SEQ ID NO: 82 - DNA, 22 bp, homo sapiens
cattagacagcagcgggcacca

SEQ ID NO: 83 - DNA, 22 bp, homo sapiens
ggcattagacagcagcgggcac

SEQ ID NO: 84 - DNA, 22 bp, homo sapiens
ggctccagggcattagacagca

SEQ ID NO: 85 - DNA, 22 bp, homo sapiens
gctcagagcggagaaagcattt

SEQ ID NO: 86 - DNA, 22 bp, homo sapiens
ggaacatttacacgtctgcgga

SEQ ID NO: 87 - DNA, 22 bp, homo sapiens
gcagacgtgtaaatgttcctgc

SEQ ID NO: 88 - DNA, 22 bp, homo sapiens
gagtctgtgtttttgcaggaac

SEQ ID NO: 89 - DNA, 22 bp, homo sapiens
gcaccaacgtacacgctccagg

SEQ ID NO: 90 - DNA, 22 bp, homo sapiens
actaaaggacaagtcaccacag

SEQ ID NO: 91 - DNA, 22 bp, homo sapiens
tatccacctcttttggcaagca

SEQ ID NO: 92 - DNA, 22 bp, homo sapiens
tgaaactcaagcaactgtcata

SEQ ID NO: 93 - DNA, 22 bp, homo sapiens
ctcacaacgtaattcacacata

SEQ ID NO: 94 - DNA, 22 bp, homo sapiens
tacttacctcacaacgtaattc

SEQ ID NO: 95 - DNA, 22 bp, homo sapiens
aacttacttacctcacaacgta

SEQ ID NO: 96 - DNA, 22 bp, homo sapiens
tcttgttttgacagtggtatta

SEQ ID NO: 97 - DNA, 22 bp, homo sapiens
gggagaaaatcaagtcgtgctg

SEQ ID NO: 98 - DNA, 22 bp, homo sapiens
tatctgaagattcaaccggttt

SEQ ID NO: 99 - DNA, 22 bp, homo sapiens
gctattcaccaaagttgaatca

SEQ ID NO: 100 - DNA, 22 bp, homo sapiens
aactttgctggccccagccgct

SEQ ID NO: 101 - DNA, 22 bp, homo sapiens
aaactgatgaccagcaacttga

SEQ ID NO: 102 - DNA, 22 bp, homo sapiens
ggggagcattacatcattatat

SEQ ID NO: 103 - DNA, 22 bp, homo sapiens
agccacttcgaagtagtgctga

SEQ ID NO: 104 - DNA, 22 bp, homo sapiens
caacttcttgattgagtgcagg

SEQ ID NO: 105 - DNA, 22 bp, homo sapiens
ttaccatgccccagattcagga

SEQ ID NO: 106 - DNA, 22 bp, homo sapiens
tcagacacctagtccttccgat

SEQ ID NO: 107 - DNA, 22 bp, homo sapiens
attggtagaaaaactttttgct

SEQ ID NO: 108 - DNA, 22 bp, homo sapiens
aactcatgtatttgctgtttta

SEQ ID NO: 109 - DNA, 22 bp, homo sapiens
aagccctgaaagcgcaagtcct

SEQ ID NO: 110 - DNA, 22 bp, homo sapiens
cagttacagtattccagcagac

SEQ ID NO: 111 - DNA, 22 bp, homo sapiens
aggttcttgtatttgagtctgc

SEQ ID NO: 112 - DNA, 22 bp, homo sapiens
atgcaatcaatattttaatgtc

SEQ ID NO: 113 - DNA, 22 bp, homo sapiens
tgattgcatctccatctcctac

SEQ ID NO: 114 - DNA, 22 bp, homo sapiens
tagtgccacatcatcaccatat

SEQ ID NO: 115 - DNA, 22 bp, homo sapiens
gagtatctctatatggtgatga

SEQ ID NO: 116 - DNA, 22 bp, homo sapiens
atacctttgactcaaagcgaca

SEQ ID NO: 117 - DNA, 22 bp, homo sapiens
ttcctgaggaagaactaaatcc

SEQ ID NO: 118 - DNA, 22 bp, homo sapiens
tctgttcactagatttgcatcc

SEQ ID NO: 119 - DNA, 22 bp, homo sapiens
gaatggagcaaaagacaattat

SEQ ID NO: 120 - DNA, 22 bp, homo sapiens
gttatgattgtgaagttaatgc

SEQ ID NO: 121 - DNA, 22 bp, homo sapiens
aacacctccgtctccttgctcc

SEQ ID NO: 122 - DNA, 22 bp, homo sapiens
tggaggccttgtccagatggga

SEQ ID NO: 123 - DNA, 22 bp, homo sapiens
tgcgactggcaatcagcttcct

SEQ ID NO: 124 - DNA, 22 bp, homo sapiens
cgactggcaatcagcttcctgc

SEQ ID NO: 125 - DNA, 22 bp, homo sapiens
gaagctgaccagcagatggaca

SEQ ID NO: 126 - DNA, 22 bp, homo sapiens
gcaatgaaaccctccaaggctt

SEQ ID NO: 127 - DNA, 22 bp, homo sapiens
aaaacatcagcaagttcatggg

SEQ ID NO: 128 - DNA, 22 bp, homo sapiens
gcaagttcatgggacttacaca

SEQ ID NO: 129 - DNA, 22 bp, homo sapiens
ggtcgcagggatgagtgaagtc

SEQ ID NO: 130 - DNA, 22 bp, homo sapiens
gcgggacttcttcatgaggatg

SEQ ID NO: 131 - DNA, 22 bp, homo sapiens
gaagtgcacggtcaccaacaga

SEQ ID NO: 132 - DNA, 22 bp, homo sapiens
acagtacggcctctgttggtga

SEQ ID NO: 133 - DNA, 22 bp, homo sapiens
tccaggtggctgacttgaggtt

SEQ ID NO: 134 - DNA, 22 bp, homo sapiens
tccacgcctgtctcaggtcttg

SEQ ID NO: 135 - DNA, 22 bp, homo sapiens
caggacagcaggggctccttgt

SEQ ID NO: 136 - DNA, 22 bp, homo sapiens
ctcatcatcatgtgtgaaccaa

SEQ ID NO: 137 - DNA, 22 bp, homo sapiens
atgtgggatgggtgctggattg

SEQ ID NO: 138 - DNA, 22 bp, homo sapiens
gccacttactacctgacccttg

SEQ ID NO: 139 - DNA, 22 bp, homo sapiens
tggccacttactacctgaccct

SEQ ID NO: 140 - DNA, 22 bp, homo sapiens
accaagggtcaggtagtaagtg

SEQ ID NO: 141 - DNA, 22 bp, homo sapiens
tagcccccatgctttgcgagca

SEQ ID NO: 142 - DNA, 22 bp, homo sapiens
gatgaccgtcccctgggtctcc

SEQ ID NO: 143 - DNA, 22 bp, homo sapiens
ctcaggacgtagttgacacaca

SEQ ID NO: 144 - DNA, 22 bp, homo sapiens
catgcttacctcaggacgtagt

SEQ ID NO: 145 - DNA, 22 bp, homo sapiens
cacatgcttacctcaggacgta

SEQ ID NO: 146 - DNA, 22 bp, homo sapiens
cagggattcagtctggtccatg

SEQ ID NO: 147 - DNA, 22 bp, homo sapiens
ggtgaataggaagttactcttc

SEQ ID NO: 148 - DNA, 22 bp, homo sapiens
atgggccacggagttgaggagc

SEQ ID NO: 149 - DNA, 22 bp, homo sapiens
ctagcccaatagccctgaagac

SEQ ID NO: 150 - DNA, 22 bp, homo sapiens
agtgattgagaagctcttcgcc

SEQ ID NO: 151 - DNA, 22 bp, homo sapiens
ggacacagaggccaaggaccaa

SEQ ID NO: 152 - DNA, 22 bp, homo sapiens
cctgatctccacagccatctac

SEQ ID NO: 153 - DNA, 22 bp, homo sapiens
cggatttcaatgagctggactt

SEQ ID NO: 154 - DNA, 22 bp, homo sapiens
tcaatgagctggacttggagac

SEQ ID NO: 155 - DNA, 22 bp, homo sapiens
gcggagaacccacagtccaccc

SEQ ID NO: 156 - DNA, 22 bp, homo sapiens
ccagtggctggaagatgtttgt

SEQ ID NO: 157 - DNA, 22 bp, homo sapiens
ttccagccactggcccctgtag

SEQ ID NO: 158 - DNA, 22 bp, homo sapiens
ctggagagcaagaagacagagc

SEQ ID NO: 159 - DNA, 22 bp, homo sapiens
gagagaggggtgctggcctggc

SEQ ID NO: 160 - DNA, 22 bp, homo sapiens
cctgccaccgtgctgtggccag

SEQ ID NO: 161 - DNA, 22 bp, homo sapiens
tctctcttccatggggggcaga

SEQ ID NO: 162 - DNA, 22 bp, homo sapiens
cacaaagtgggccgtcggggat

SEQ ID NO: 163 - DNA, 22 bp, homo sapiens
ggagagggctaccatggccgga

SEQ ID NO: 164 - DNA, 22 bp, homo sapiens
ctcaggtcctggaaggcttgct

SEQ ID NO: 165 - DNA, 22 bp, homo sapiens
ctcccagggggacccacctggt

SEQ ID NO: 166 - DNA, 22 bp, homo sapiens
tgccggacaagccactgagcgc

SEQ ID NO: 167 - DNA, 22 bp, homo sapiens
ttccccccacagtgctacgcca

SEQ ID NO: 168 - DNA, 22 bp, homo sapiens
ctgtagtcctggtactgggtgg

SEQ ID NO: 169 - DNA, 22 bp, homo sapiens
tgggctgacgacaggctgtagt

SEQ ID NO: 170 - DNA, 22 bp, homo sapiens
tccttgcaggagcgtggagctt

SEQ ID NO: 171 - DNA, 22 bp, homo sapiens
gactgtgctgaagtattcaaat

SEQ ID NO: 172 - DNA, 22 bp, homo sapiens
ctgtgctgaagtattcaaatca

SEQ ID NO: 173 - DNA, 22 bp, homo sapiens
tggtgtgtcctgatttgaatac

SEQ ID NO: 174 - DNA, 22 bp, homo sapiens
gccattcgtggtgtgtcctgat

SEQ ID NO: 175 - DNA, 22 bp, homo sapiens
atcaggacacaccacgaatggc

SEQ ID NO: 176 - DNA, 22 bp, homo sapiens
ctaatcagcaacgctatgtgct

SEQ ID NO: 177 - DNA, 22 bp, homo sapiens
aatcagcaacgctatgtgctta

SEQ ID NO: 178 - DNA, 22 bp, homo sapiens
ttcccagtctttaaggtgtatt

SEQ ID NO: 179 - DNA, 22 bp, homo sapiens
tcttcacttgagagatagaaat

SEQ ID NO: 180 - DNA, 22 bp, homo sapiens
catcagccaaccaggaaatgat

SEQ ID NO: 181 - DNA, 22 bp, homo sapiens
ctgttagcatttgtgaacattt

SEQ ID NO: 182 - DNA, 22 bp, homo sapiens
tgtggtccttccaacttgaacg

SEQ ID NO: 183 - DNA, 22 bp, homo sapiens
cggaatgtactatccacagagg

SEQ ID NO: 184 - DNA, 22 bp, homo sapiens
ttatttgtgttctgcctctgtg

SEQ ID NO: 185 - DNA, 22 bp, homo sapiens
acaaataagttcaacggcatta

SEQ ID NO: 186 - DNA, 22 bp, homo sapiens
agcgaatagcctgagcctttcc

SEQ ID NO: 187 - DNA, 20 bp, homo sapiens
cagctgaccagtcgcgctga

SEQ ID NO: 188 - DNA, 20 bp, homo sapiens
gtggtagctggggctggggg

SEQ ID NO: 189 - DNA, 20 bp, homo sapiens
gaggtggtagctggggctgg

SEQ ID NO: 190 - DNA, 20 bp, homo sapiens
ggaggtggtagctggggctg

SEQ ID NO: 191 - DNA, 20 bp, homo sapiens
aggaggtggtagctggggct

SEQ ID NO: 192 - DNA, 20 bp, homo sapiens
gaggaggtggtagctggggc

SEQ ID NO: 193 - DNA, 20 bp, homo sapiens
cggggaggaggtggtagctg

SEQ ID NO: 194 - DNA, 20 bp, homo sapiens
cccagctaccacctcctccc

SEQ ID NO: 195 - DNA, 20 bp, homo sapiens
ccggggaggaggtggtagct

SEQ ID NO: 196 - DNA, 20 bp, homo sapiens
gccggggaggaggtggtagc

SEQ ID NO: 197 - DNA, 20 bp, homo sapiens
gctaccacctcctccccggc

SEQ ID NO: 198 - DNA, 20 bp, homo sapiens
accacctcctccccggccgg

SEQ ID NO: 199 - DNA, 20 bp, homo sapiens
gccgccggccggggaggagg

SEQ ID NO: 200 - DNA, 20 bp, homo sapiens
acctcctccccggccggcgg

SEQ ID NO: 201 - DNA, 20 bp, homo sapiens
tccgccgccggccggggagg

SEQ ID NO: 202 - DNA, 20 bp, homo sapiens
ctgtccgccgccggccgggg

SEQ ID NO: 203 - DNA, 20 bp, homo sapiens
ccccggccggcggcggacag

SEQ ID NO: 204 - DNA, 20 bp, homo sapiens
ccactgtccgccgccggccg

SEQ ID NO: 205 - DNA, 20 bp, homo sapiens
tccactgtccgccgccggcc

SEQ ID NO: 206 - DNA, 20 bp, homo sapiens
gtccactgtccgccgccggc

SEQ ID NO: 207 - DNA, 20 bp, homo sapiens
ccggcggcggacagtggacg

SEQ ID NO: 208 - DNA, 20 bp, homo sapiens
ccgcgtccactgtccgccgc

SEQ ID NO: 209 - DNA, 20 bp, homo sapiens
gcggcggacagtggacgcgg

SEQ ID NO: 210 - DNA, 20 bp, homo sapiens
gtggacgcggcggcgagccg

SEQ ID NO: 211 - DNA, 20 bp, homo sapiens
tggacgcggcggcgagccgc

SEQ ID NO: 212 - DNA, 20 bp, homo sapiens
cgcggcggcgagccgcgggc

SEQ ID NO: 213 - DNA, 20 bp, homo sapiens
gcggcggcgagccgcgggca

SEQ ID NO: 214 - DNA, 20 bp, homo sapiens
cggcggcgagccgcgggcag

SEQ ID NO: 215 - DNA, 20 bp, homo sapiens
ggcgagccgcgggcaggggc

SEQ ID NO: 216 - DNA, 20 bp, homo sapiens
cgggctccggcccctgcccg

SEQ ID NO: 217 - DNA, 20 bp, homo sapiens
caggggccggagcccgcgcc

SEQ ID NO: 218 - DNA, 20 bp, homo sapiens
gggccggagcccgcgcccgg

SEQ ID NO: 219 - DNA, 20 bp, homo sapiens
ccggagcccgcgcccggagg

SEQ ID NO: 220 - DNA, 20 bp, homo sapiens
ccgcctccgggcgcgggctc

SEQ ID NO: 221 - DNA, 20 bp, homo sapiens
cggagcccgcgcccggaggc

SEQ ID NO: 222 - DNA, 20 bp, homo sapiens
ggagcccgcgcccggaggcg

SEQ ID NO: 223 - DNA, 20 bp, homo sapiens
gcccgcgcccggaggcgggg

SEQ ID NO: 224 - DNA, 20 bp, homo sapiens
tccaccccgcctccgggcgc

SEQ ID NO: 225 - DNA, 20 bp, homo sapiens
ctccaccccgcctccgggcg

SEQ ID NO: 226 - DNA, 20 bp, homo sapiens
cgcgcccggaggcggggtgg

SEQ ID NO: 227 - DNA, 20 bp, homo sapiens
gcgcccggaggcggggtgga

SEQ ID NO: 228 - DNA, 20 bp, homo sapiens
cgcccggaggcggggtggag

SEQ ID NO: 229 - DNA, 20 bp, homo sapiens
gcccggaggcggggtggagg

SEQ ID NO: 230 - DNA, 20 bp, homo sapiens
accccctccaccccgcctcc

SEQ ID NO: 231 - DNA, 20 bp, homo sapiens
gaccccctccaccccgcctc

SEQ ID NO: 232 - DNA, 20 bp, homo sapiens
ggaggcggggtggagggggt

SEQ ID NO: 233 - DNA, 20 bp, homo sapiens
gaggcggggtggagggggtc

SEQ ID NO: 234 - DNA, 20 bp, homo sapiens
aggcggggtggagggggtcg

SEQ ID NO: 235 - DNA, 20 bp, homo sapiens
gtggagggggtcggggctcg

SEQ ID NO: 236 - DNA, 20 bp, homo sapiens
gaaacttttcgtccaacttc

SEQ ID NO: 237 - DNA, 20 bp, homo sapiens
aaacttttcgtccaacttct

SEQ ID NO: 238 - DNA, 20 bp, homo sapiens
agcgagaacagcccagaagt

SEQ ID NO: 239 - DNA, 20 bp, homo sapiens
cttctgggctgttctcgctt

SEQ ID NO: 240 - DNA, 20 bp, homo sapiens
ctgggctgttctcgcttcgg

SEQ ID NO: 241 - DNA, 20 bp, homo sapiens
ttctcgcttcggaggagccg

SEQ ID NO: 242 - DNA, 20 bp, homo sapiens
cggaggagccgtggtccgcg

SEQ ID NO: 243 - DNA, 20 bp, homo sapiens
ggaggagccgtggtccgcgc

SEQ ID NO: 244 - DNA, 20 bp, homo sapiens
gaggagccgtggtccgcgcg

SEQ ID NO: 245 - DNA, 20 bp, homo sapiens
aggagccgtggtccgcgcgg

SEQ ID NO: 246 - DNA, 20 bp, homo sapiens
ggcttcccccgcgcggacca

SEQ ID NO: 247 - DNA, 20 bp, homo sapiens
tcggctcggcttcccccgcg

SEQ ID NO: 248 - DNA, 20 bp, homo sapiens
gcgggggaagccgagccgag

SEQ ID NO: 249 - DNA, 20 bp, homo sapiens
tctcgcggctccgctcggct

SEQ ID NO: 250 - DNA, 20 bp, homo sapiens
gcacttctcgcggctccgct

SEQ ID NO: 251 - DNA, 20 bp, homo sapiens
agccgcgagaagtgctagct

SEQ ID NO: 252 - DNA, 20 bp, homo sapiens
gccgcgagaagtgctagctc

SEQ ID NO: 253 - DNA, 20 bp, homo sapiens
gcccgagctagcacttctcg

SEQ ID NO: 254 - DNA, 20 bp, homo sapiens
cgagaagtgctagctcgggc

SEQ ID NO: 255 - DNA, 20 bp, homo sapiens
gagaagtgctagctcgggcc

SEQ ID NO: 256 - DNA, 20 bp, homo sapiens
aagtgctagctcgggccggg

SEQ ID NO: 257 - DNA, 20 bp, homo sapiens
gggccgggaggagccgcagc

SEQ ID NO: 258 - DNA, 20 bp, homo sapiens
ccgggaggagccgcagccgg

SEQ ID NO: 259 - DNA, 20 bp, homo sapiens
cctccggctgcggctcctcc

SEQ ID NO: 260 - DNA, 20 bp, homo sapiens
ggaggagccgcagccggagg

SEQ ID NO: 261 - DNA, 20 bp, homo sapiens
gaggagccgcagccggagga

SEQ ID NO: 262 - DNA, 20 bp, homo sapiens
aggagccgcagccggaggag

SEQ ID NO: 263 - DNA, 20 bp, homo sapiens
ggagccgcagccggaggagg

SEQ ID NO: 264 - DNA, 20 bp, homo sapiens
gccgcagccggaggaggggg

SEQ ID NO: 265 - DNA, 20 bp, homo sapiens
tcctccccctcctccggctg

SEQ ID NO: 266 - DNA, 20 bp, homo sapiens
gcagccggaggagggggagg

SEQ ID NO: 267 - DNA, 20 bp, homo sapiens
tcttcctcctccccctcctc

SEQ ID NO: 268 - DNA, 20 bp, homo sapiens
gaagagaaggaagaggagag

SEQ ID NO: 269 - DNA, 20 bp, homo sapiens
aagagaaggaagaggagagg

SEQ ID NO: 270 - DNA, 20 bp, homo sapiens
aagaggagagggggccgcag

SEQ ID NO: 271 - DNA, 20 bp, homo sapiens
agggggccgcagtggcgact

SEQ ID NO: 272 - DNA, 20 bp, homo sapiens
cgagcgccgagtcgccactg

SEQ ID NO: 273 - DNA, 20 bp, homo sapiens
cgcagtggcgactcggcgct

SEQ ID NO: 274 - DNA, 20 bp, homo sapiens
gcgactcggcgctcggaagc

SEQ ID NO: 275 - DNA, 20 bp, homo sapiens
cgactcggcgctcggaagcc

SEQ ID NO: 276 - DNA, 20 bp, homo sapiens
gcgctcggaagccgggctca

SEQ ID NO: 277 - DNA, 20 bp, homo sapiens
tcggaagccgggctcatgga

SEQ ID NO: 278 - DNA, 20 bp, homo sapiens
cggaagccgggctcatggac

SEQ ID NO: 279 - DNA, 20 bp, homo sapiens
gccgggctcatggacgggtg

SEQ ID NO: 280 - DNA, 20 bp, homo sapiens
gcctcacccgtccatgagcc

SEQ ID NO: 281 - DNA, 20 bp, homo sapiens
gggctcatggacgggtgagg

SEQ ID NO: 282 - DNA, 20 bp, homo sapiens
ctcatggacgggtgaggcgg

SEQ ID NO: 283 - DNA, 20 bp, homo sapiens
tccagccgcgcgcgctcccc

SEQ ID NO: 284 - DNA, 20 bp, homo sapiens
gcctggggagcgcgcgcggc

SEQ ID NO: 285 - DNA, 20 bp, homo sapiens
cagggcctggggagcgcgcg

SEQ ID NO: 286 - DNA, 20 bp, homo sapiens
cgcgcgcgctccccaggccc

SEQ ID NO: 287 - DNA, 20 bp, homo sapiens
gcgctccccaggccctggcc

SEQ ID NO: 288 - DNA, 20 bp, homo sapiens
cgctccccaggccctggccc

SEQ ID NO: 289 - DNA, 20 bp, homo sapiens
gaggcccgggccagggcctg

SEQ ID NO: 290 - DNA, 20 bp, homo sapiens
cgaggcccgggccagggcct

SEQ ID NO: 291 - DNA, 20 bp, homo sapiens
ccaggccctggcccgggcct

SEQ ID NO: 292 - DNA, 20 bp, homo sapiens
ccgaggcccgggccagggcc

SEQ ID NO: 293 - DNA, 20 bp, homo sapiens
caggccctggcccgggcctc

SEQ ID NO: 294 - DNA, 20 bp, homo sapiens
ccctggcccgggcctcgggc

SEQ ID NO: 295 - DNA, 20 bp, homo sapiens
ccggcccgaggcccgggcca

SEQ ID NO: 296 - DNA, 20 bp, homo sapiens
cctggcccgggcctcgggcc

SEQ ID NO: 297 - DNA, 20 bp, homo sapiens
cccggcccgaggcccgggcc

SEQ ID NO: 298 - DNA, 20 bp, homo sapiens
ctggcccgggcctcgggccg

SEQ ID NO: 299 - DNA, 20 bp, homo sapiens
gcccgggcctcgggccgggg

SEQ ID NO: 300 - DNA, 20 bp, homo sapiens
tcctccccggcccgaggccc

SEQ ID NO: 301 - DNA, 20 bp, homo sapiens
ttcctccccggcccgaggcc

SEQ ID NO: 302 - DNA, 20 bp, homo sapiens
tactcttcctccccggcccg

SEQ ID NO: 303 - DNA, 20 bp, homo sapiens
ggcgagctactcttcctccc

SEQ ID NO: 304 - DNA, 20 bp, homo sapiens
ggaggaagagtagctcgccg

SEQ ID NO: 305 - DNA, 20 bp, homo sapiens
agtagctcgccgaggcgccg

SEQ ID NO: 306 - DNA, 20 bp, homo sapiens
cgccgaggcgccgaggagag

SEQ ID NO: 307 - DNA, 20 bp, homo sapiens
gccgaggcgccgaggagagc

SEQ ID NO: 308 - DNA, 20 bp, homo sapiens
gcccgctctcctcggcgcct

SEQ ID NO: 309 - DNA, 20 bp, homo sapiens
gtggggcggcccgctctcct

SEQ ID NO: 310 - DNA, 20 bp, homo sapiens
ggccgccccacagcccgagc

SEQ ID NO: 311 - DNA, 20 bp, homo sapiens
ctccggctcgggctgtgggg

SEQ ID NO: 312 - DNA, 20 bp, homo sapiens
ccccacagcccgagccggag

SEQ ID NO: 313 - DNA, 20 bp, homo sapiens
cctctccggctcgggctgtg

SEQ ID NO: 314 - DNA, 20 bp, homo sapiens
cccacagcccgagccggaga

SEQ ID NO: 315 - DNA, 20 bp, homo sapiens
ccctctccggctcgggctgt

SEQ ID NO: 316 - DNA, 20 bp, homo sapiens
tccctctccggctcgggctg

SEQ ID NO: 317 - DNA, 20 bp, homo sapiens
tcgcgctccctctccggctc

SEQ ID NO: 318 - DNA, 20 bp, homo sapiens
ctcgcgctccctctccggct

SEQ ID NO: 319 - DNA, 20 bp, homo sapiens
cgcggctcgcgctccctctc

SEQ ID NO: 320 - DNA, 20 bp, homo sapiens
agagggagcgcgagccgcgc

SEQ ID NO: 321 - DNA, 20 bp, homo sapiens
cgagccgcgccggccccggt

SEQ ID NO: 322 - DNA, 20 bp, homo sapiens
gagccgcgccggccccggtc

SEQ ID NO: 323 - DNA, 20 bp, homo sapiens
aggcccgaccggggccggcg

SEQ ID NO: 324 - DNA, 20 bp, homo sapiens
ttcggaggcccgaccggggc

SEQ ID NO: 325 - DNA, 20 bp, homo sapiens
tggtttcggaggcccgaccg

SEQ ID NO: 326 - DNA, 20 bp, homo sapiens
atggtttcggaggcccgacc

SEQ ID NO: 327 - DNA, 20 bp, homo sapiens
catggtttcggaggcccgac

SEQ ID NO: 328 - DNA, 20 bp, homo sapiens
cagaaagttcatggtttcgg

SEQ ID NO: 329 - DNA, 20 bp, homo sapiens
cagcagaaagttcatggttt

SEQ ID NO: 330 - DNA, 20 bp, homo sapiens
ccatgaactttctgctgtct

SEQ ID NO: 331 - DNA, 20 bp, homo sapiens
ccaagacagcagaaagttca

SEQ ID NO: 332 - DNA, 20 bp, homo sapiens
catgaactttctgctgtctt

SEQ ID NO: 333 - DNA, 20 bp, homo sapiens
ttctgctgtcttgggtgcat

SEQ ID NO: 334 - DNA, 20 bp, homo sapiens
ggaggtagagcagcaaggca

SEQ ID NO: 335 - DNA, 20 bp, homo sapiens
atggtggaggtagagcagca

SEQ ID NO: 336 - DNA, 20 bp, homo sapiens
gctctacctccaccatgcca

SEQ ID NO: 337 - DNA, 20 bp, homo sapiens
cgcttaccttggcatggtgg

SEQ ID NO: 338 - DNA, 20 bp, homo sapiens
gaccgcttaccttggcatgg

SEQ ID NO: 339 - DNA, 20 bp, homo sapiens
cacgaccgcttaccttggca

SEQ ID NO: 340 - DNA, 20 bp, homo sapiens
tttctgtcctcagtggtccc

SEQ ID NO: 341 - DNA, 20 bp, homo sapiens
ggtgcagcctgggaccactg

SEQ ID NO: 342 - DNA, 20 bp, homo sapiens
gtggtcccaggctgcaccca

SEQ ID NO: 343 - DNA, 20 bp, homo sapiens
ttctgccatgggtgcagcct

SEQ ID NO: 344 - DNA, 20 bp, homo sapiens
cttctgccatgggtgcagcc

SEQ ID NO: 345 - DNA, 20 bp, homo sapiens
caggctgcacccatggcaga

SEQ ID NO: 346 - DNA, 20 bp, homo sapiens
gctgcacccatggcagaagg

SEQ ID NO: 347 - DNA, 20 bp, homo sapiens
gcacccatggcagaaggagg

SEQ ID NO: 348 - DNA, 20 bp, homo sapiens
cacccatggcagaaggagga

SEQ ID NO: 349 - DNA, 20 bp, homo sapiens
tgccctcctccttctgccat

SEQ ID NO: 350 - DNA, 20 bp, homo sapiens
ctgccctcctccttctgcca

SEQ ID NO: 351 - DNA, 20 bp, homo sapiens
ggagggcagaatcatcacga

SEQ ID NO: 352 - DNA, 20 bp, homo sapiens
tcatgcagtggtgaagttca

SEQ ID NO: 353 - DNA, 20 bp, homo sapiens
ctgccatccaatcgagaccc

SEQ ID NO: 354 - DNA, 20 bp, homo sapiens
ccatccaatcgagaccctgg

SEQ ID NO: 355 - DNA, 20 bp, homo sapiens
ccaccagggtctcgattgga

SEQ ID NO: 356 - DNA, 20 bp, homo sapiens
atgtccaccagggtctcgat

SEQ ID NO: 357 - DNA, 20 bp, homo sapiens
gaccctggtggacatcttcc

SEQ ID NO: 358 - DNA, 20 bp, homo sapiens
ctcctggaagatgtccacca

SEQ ID NO: 359 - DNA, 20 bp, homo sapiens
actcctggaagatgtccacc

SEQ ID NO: 360 - DNA, 20 bp, homo sapiens
cgatctcatcagggtactcc

SEQ ID NO: 361 - DNA, 20 bp, homo sapiens
agatgtactcgatctcatca

SEQ ID NO: 362 - DNA, 20 bp, homo sapiens
aagatgtactcgatctcatc

SEQ ID NO: 363 - DNA, 20 bp, homo sapiens
cgcatcaggggcacacagga

SEQ ID NO: 364 - DNA, 20 bp, homo sapiens
gcatcgcatcaggggcacac

SEQ ID NO: 365 - DNA, 20 bp, homo sapiens
tgtgtgcccctgatgcgatg

SEQ ID NO: 366 - DNA, 20 bp, homo sapiens
gtgtgcccctgatgcgatgc

SEQ ID NO: 367 - DNA, 20 bp, homo sapiens
tgtgcccctgatgcgatgcg

SEQ ID NO: 368 - DNA, 20 bp, homo sapiens
gtgcccctgatgcgatgcgg

SEQ ID NO: 369 - DNA, 20 bp, homo sapiens
cagcccccgcatcgcatcag

SEQ ID NO: 370 - DNA, 20 bp, homo sapiens
gcagcccccgcatcgcatca

SEQ ID NO: 371 - DNA, 20 bp, homo sapiens
agcagcccccgcatcgcatc

SEQ ID NO: 372 - DNA, 20 bp, homo sapiens
cgggggctgctgcaatgacg

SEQ ID NO: 373 - DNA, 20 bp, homo sapiens
gggggctgctgcaatgacga

SEQ ID NO: 374 - DNA, 20 bp, homo sapiens
ctgctgcaatgacgagggcc

SEQ ID NO: 375 - DNA, 20 bp, homo sapiens
cctggagtgtgtgcccactg

SEQ ID NO: 376 - DNA, 20 bp, homo sapiens
cctcagtgggcacacactcc

SEQ ID NO: 377 - DNA, 20 bp, homo sapiens
gtgatgttggactcctcagt

SEQ ID NO: 378 - DNA, 20 bp, homo sapiens
ggtgatgttggactcctcag

SEQ ID NO: 379 - DNA, 20 bp, homo sapiens
ggagtccaacatcaccatgc

SEQ ID NO: 380 - DNA, 20 bp, homo sapiens
gtccaacatcaccatgcagg

SEQ ID NO: 381 - DNA, 20 bp, homo sapiens
tccaacatcaccatgcaggt

SEQ ID NO: 382 - DNA, 20 bp, homo sapiens
gcccacctgcatggtgatgt

SEQ ID NO: 383 - DNA, 20 bp, homo sapiens
cccaaagatgcccacctgca

SEQ ID NO: 384 - DNA, 20 bp, homo sapiens
tccttcctttccagattatg

SEQ ID NO: 385 - DNA, 20 bp, homo sapiens
gaggtttgatccgcataatc

SEQ ID NO: 386 - DNA, 20 bp, homo sapiens
atgcggatcaaacctcacca

SEQ ID NO: 387 - DNA, 20 bp, homo sapiens
cctcaccaaggccagcacat

SEQ ID NO: 388 - DNA, 20 bp, homo sapiens
cctatgtgctggccttggtg

SEQ ID NO: 389 - DNA, 20 bp, homo sapiens
tctctcctatgtgctggcct

SEQ ID NO: 390 - DNA, 20 bp, homo sapiens
agctcatctctcctatgtgc

SEQ ID NO: 391 - DNA, 20 bp, homo sapiens
attcacatttgttgtgctgt

SEQ ID NO: 392 - DNA, 20 bp, homo sapiens
agcacaacaaatgtgaatgc

SEQ ID NO: 393 - DNA, 20 bp, homo sapiens
aacaaatgtgaatgcaggtg

SEQ ID NO: 394 - DNA, 20 bp, homo sapiens
tgtcttgctctatctttctt

SEQ ID NO: 395 - DNA, 20 bp, homo sapiens
ttttccagaaaatcagttcg

SEQ ID NO: 396 - DNA, 20 bp, homo sapiens
ctttcctcgaactgattttc

SEQ ID NO: 397 - DNA, 20 bp, homo sapiens
cagaaaatcagttcgaggaa

SEQ ID NO: 398 - DNA, 20 bp, homo sapiens
agaaaatcagttcgaggaaa

SEQ ID NO: 399 - DNA, 20 bp, homo sapiens
atcagttcgaggaaagggaa

SEQ ID NO: 400 - DNA, 20 bp, homo sapiens
tcagttcgaggaaagggaaa

SEQ ID NO: 401 - DNA, 20 bp, homo sapiens
cagttcgaggaaagggaaag

SEQ ID NO: 402 - DNA, 20 bp, homo sapiens
aacgaaagcgcaagaaatcc

SEQ ID NO: 403 - DNA, 20 bp, homo sapiens
agaaatcccggtataagtcc

SEQ ID NO: 404 - DNA, 20 bp, homo sapiens
cacgctccaggacttatacc

SEQ ID NO: 405 - DNA, 20 bp, homo sapiens
acacgctccaggacttatac

SEQ ID NO: 406 - DNA, 20 bp, homo sapiens
aagtcctggagcgtgtacgt

SEQ ID NO: 407 - DNA, 20 bp, homo sapiens
ggcaccaacgtacacgctcc

SEQ ID NO: 408 - DNA, 20 bp, homo sapiens
cccgctgctgtctaatgccc

SEQ ID NO: 409 - DNA, 20 bp, homo sapiens
ccagggcattagacagcagc

SEQ ID NO: 410 - DNA, 20 bp, homo sapiens
tccagggcattagacagcag

SEQ ID NO: 411 - DNA, 20 bp, homo sapiens
ctaatgccctggagcctccc

SEQ ID NO: 412 - DNA, 20 bp, homo sapiens
tgggggccagggaggctcca

SEQ ID NO: 413 - DNA, 20 bp, homo sapiens
ctgggggccagggaggctcc

SEQ ID NO: 414 - DNA, 20 bp, homo sapiens
ggttgtactgggggccaggg

SEQ ID NO: 415 - DNA, 20 bp, homo sapiens
ggaggttgtactgggggcca

SEQ ID NO: 416 - DNA, 20 bp, homo sapiens
cggaggttgtactgggggcc

SEQ ID NO: 417 - DNA, 20 bp, homo sapiens
gcaggcggaggttgtactgg

SEQ ID NO: 418 - DNA, 20 bp, homo sapiens
ttgcctttttgcagtccctg

SEQ ID NO: 419 - DNA, 20 bp, homo sapiens
tgcctttttgcagtccctgt

SEQ ID NO: 420 - DNA, 20 bp, homo sapiens
cgctctgagcaaggcccaca

SEQ ID NO: 421 - DNA, 20 bp, homo sapiens
cctgtgggccttgctcagag

SEQ ID NO: 422 - DNA, 20 bp, homo sapiens
ccgctctgagcaaggcccac

SEQ ID NO: 423 - DNA, 20 bp, homo sapiens
tgctttctccgctctgagca

SEQ ID NO: 424 - DNA, 20 bp, homo sapiens
caggaacatttacacgtctg

SEQ ID NO: 425 - DNA, 20 bp, homo sapiens
acgcgagtctgtgtttttgc

SEQ ID NO: 426 - DNA, 20 bp, homo sapiens
aaacacagactcgcgttgca

SEQ ID NO: 427 - DNA, 20 bp, homo sapiens
cagactcgcgttgcaaggcg

SEQ ID NO: 428 - DNA, 20 bp, homo sapiens
agttaaacgaacgtacttgc

SEQ ID NO: 429 - DNA, 20 bp, homo sapiens
aaacgaacgtacttgcaggt

SEQ ID NO: 430 - DNA, 20 bp, homo sapiens
ccctcagatgtgacaagccg

SEQ ID NO: 431 - DNA, 20 bp, homo sapiens
gcctcggcttgtcacatctg

SEQ ID NO: 432 - DNA, 20 bp, homo sapiens
tcagatgtgacaagccgagg

SEQ ID NO: 433 - DNA, 20 bp, homo sapiens
acaagccgaggcggtgagcc

SEQ ID NO: 434 - DNA, 20 bp, homo sapiens
gccgaggcggtgagccgggc

SEQ ID NO: 435 - DNA, 20 bp, homo sapiens
tcctgcccggctcaccgcct

SEQ ID NO: 436 - DNA, 20 bp, homo sapiens
tttaaatgagctcccaatgt

SEQ ID NO: 437 - DNA, 20 bp, homo sapiens
gagctcccaatgtcggagtt

SEQ ID NO: 438 - DNA, 20 bp, homo sapiens
gttttccaaactccgacatt

SEQ ID NO: 439 - DNA, 20 bp, homo sapiens
tgttttccaaactccgacat

SEQ ID NO: 440 - DNA, 20 bp, homo sapiens
aaatttgtctttttaaaaga

SEQ ID NO: 441 - DNA, 20 bp, homo sapiens
gtctttttaaaagaaggtct

SEQ ID NO: 442 - DNA, 20 bp, homo sapiens
aaactcaaaacctgaagaat

SEQ ID NO: 443 - DNA, 20 bp, homo sapiens
ctgatttcttccaattcttc

SEQ ID NO: 444 - DNA, 20 bp, homo sapiens
gaagaaatcagaatagaaaa

SEQ ID NO: 445 - DNA, 20 bp, homo sapiens
aagaaatcagaatagaaaat

SEQ ID NO: 446 - DNA, 20 bp, homo sapiens
atcagaatagaaaatgggta

SEQ ID NO: 447 - DNA, 20 bp, homo sapiens
ctcgagatgcagccagatct

SEQ ID NO: 448 - DNA, 20 bp, homo sapiens
ttctttacttcgccgagatc

SEQ ID NO: 449 - DNA, 20 bp, homo sapiens
gaactcacattatgtggaag

SEQ ID NO: 450 - DNA, 20 bp, homo sapiens
agatgcgaactcacattatg

SEQ ID NO: 451 - DNA, 20 bp, homo sapiens
tgtgagttcgcatcttgata

SEQ ID NO: 452 - DNA, 20 bp, homo sapiens
ttgataaggcctctgtgatg

SEQ ID NO: 453 - DNA, 20 bp, homo sapiens
gatggtaagcctcatcacag

SEQ ID NO: 454 - DNA, 20 bp, homo sapiens
ccatcagctatttgcgtgtg

SEQ ID NO: 455 - DNA, 20 bp, homo sapiens
cctcacacgcaaatagctga

SEQ ID NO: 456 - DNA, 20 bp, homo sapiens
tttgcgtgtgaggaaacttc

SEQ ID NO: 457 - DNA, 20 bp, homo sapiens
gtgaggaaacttctggatgc

SEQ ID NO: 458 - DNA, 20 bp, homo sapiens
tgtgccctttttaggtgatt

SEQ ID NO: 459 - DNA, 20 bp, homo sapiens
ttgcttttatttgaaagcct

SEQ ID NO: 460 - DNA, 20 bp, homo sapiens
ttttatttgaaagccttgga

SEQ ID NO: 461 - DNA, 20 bp, homo sapiens
agccttggatggttttgtta

SEQ ID NO: 462 - DNA, 20 bp, homo sapiens
aaccataacaaaaccatcca

SEQ ID NO: 463 - DNA, 20 bp, homo sapiens
gttatggttctcacagatga

SEQ ID NO: 464 - DNA, 20 bp, homo sapiens
tgataatgtgaacaaataca

SEQ ID NO: 465 - DNA, 20 bp, homo sapiens
gataatgtgaacaaatacat

SEQ ID NO: 466 - DNA, 20 bp, homo sapiens
caaatacatgggattaactc

SEQ ID NO: 467 - DNA, 20 bp, homo sapiens
tgtttacagtttgaactaac

SEQ ID NO: 468 - DNA, 20 bp, homo sapiens
tactcatccatgtgaccatg

SEQ ID NO: 469 - DNA, 20 bp, homo sapiens
ctcatttcctcatggtcaca

SEQ ID NO: 470 - DNA, 20 bp, homo sapiens
gcatttctctcatttcctca

SEQ ID NO: 471 - DNA, 20 bp, homo sapiens
gaaatgcttacacacagaaa

SEQ ID NO: 472 - DNA, 20 bp, homo sapiens
ttcattaggccttgtgaaaa

SEQ ID NO: 473 - DNA, 20 bp, homo sapiens
tcattaggccttgtgaaaaa

SEQ ID NO: 474 - DNA, 20 bp, homo sapiens
gttctttaccctttttcaca

SEQ ID NO: 475 - DNA, 20 bp, homo sapiens
aagtgtaccctaactagccg

SEQ ID NO: 476 - DNA, 20 bp, homo sapiens
agttcttcctcggctagtta

SEQ ID NO: 477 - DNA, 20 bp, homo sapiens
tagttcttcctcggctagtt

SEQ ID NO: 478 - DNA, 20 bp, homo sapiens
ttatgttcatagttcttcct

SEQ ID NO: 479 - DNA, 20 bp, homo sapiens
tgaacataaagtctgcaaca

SEQ ID NO: 480 - DNA, 20 bp, homo sapiens
cataaagtctgcaacatgga

SEQ ID NO: 481 - DNA, 20 bp, homo sapiens
acacaggtattgcactgcac

SEQ ID NO: 482 - DNA, 20 bp, homo sapiens
tggtatcatatacgtgaatg

SEQ ID NO: 483 - DNA, 20 bp, homo sapiens
acactgaggttggttactgt

SEQ ID NO: 484 - DNA, 20 bp, homo sapiens
aacagtaaccaacctcagtg

SEQ ID NO: 485 - DNA, 20 bp, homo sapiens
acagtaaccaacctcagtgt

SEQ ID NO: 486 - DNA, 20 bp, homo sapiens
tcttatacccacactgaggt

SEQ ID NO: 487 - DNA, 20 bp, homo sapiens
ggtttcttatacccacactg

SEQ ID NO: 488 - DNA, 20 bp, homo sapiens
gaaaccacctatgacctgct

SEQ ID NO: 489 - DNA, 20 bp, homo sapiens
agcaccaagcaggtcatagg

SEQ ID NO: 490 - DNA, 20 bp, homo sapiens
atcagcaccaagcaggtcat

SEQ ID NO: 491 - DNA, 20 bp, homo sapiens
ttcacaaatcagcaccaagc

SEQ ID NO: 492 - DNA, 20 bp, homo sapiens
atatttgatgggtgaggaat

SEQ ID NO: 493 - DNA, 20 bp, homo sapiens
aatatttgatgggtgaggaa

SEQ ID NO: 494 - DNA, 20 bp, homo sapiens
atttcaatatttgatgggtg

SEQ ID NO: 495 - DNA, 20 bp, homo sapiens
aaggaatttcaatatttgat

SEQ ID NO: 496 - DNA, 20 bp, homo sapiens
aaaggaatttcaatatttga

SEQ ID NO: 497 - DNA, 20 bp, homo sapiens
aggaaagtcttgctatctaa

SEQ ID NO: 498 - DNA, 20 bp, homo sapiens
tttcctcagtcgacacagcc

SEQ ID NO: 499 - DNA, 20 bp, homo sapiens
tatccaggctgtgtcgactg

SEQ ID NO: 500 - DNA, 20 bp, homo sapiens
aataagaaaatttcatatcc

SEQ ID NO: 501 - DNA, 20 bp, homo sapiens
aattttcttattgtgatgaa

SEQ ID NO: 502 - DNA, 20 bp, homo sapiens
taacagaattaccgaattga

SEQ ID NO: 503 - DNA, 20 bp, homo sapiens
aacagaattaccgaattgat

SEQ ID NO: 504 - DNA, 20 bp, homo sapiens
tggctcatatcccatcaatt

SEQ ID NO: 505 - DNA, 20 bp, homo sapiens
tatgagccagaagaactttt

SEQ ID NO: 506 - DNA, 20 bp, homo sapiens
gagcggcctaaaagttcttc

SEQ ID NO: 507 - DNA, 20 bp, homo sapiens
gataatattcataaattgag

SEQ ID NO: 508 - DNA, 20 bp, homo sapiens
ttatgaatattatcatgctt

SEQ ID NO: 509 - DNA, 20 bp, homo sapiens
cttactatcatgatgagttt

SEQ ID NO: 510 - DNA, 20 bp, homo sapiens
tcccccctagtgtttactaa

SEQ ID NO: 511 - DNA, 20 bp, homo sapiens
ttgtcctttagtaaacacta

SEQ ID NO: 512 - DNA, 20 bp, homo sapiens
cttgtcctttagtaaacact

SEQ ID NO: 513 - DNA, 20 bp, homo sapiens
actaaaggacaagtcaccac

SEQ ID NO: 514 - DNA, 20 bp, homo sapiens
aagtcaccacaggacagtac

SEQ ID NO: 515 - DNA, 20 bp, homo sapiens
aagcatcctgtactgtcctg

SEQ ID NO: 516 - DNA, 20 bp, homo sapiens
tacaggatgcttgccaaaag

SEQ ID NO: 517 - DNA, 20 bp, homo sapiens
aggatgcttgccaaaagagg

SEQ ID NO: 518 - DNA, 20 bp, homo sapiens
ccaaaagaggtggatatgtc

SEQ ID NO: 519 - DNA, 20 bp, homo sapiens
ccagacatatccacctcttt

SEQ ID NO: 520 - DNA, 20 bp, homo sapiens
caaaagaggtggatatgtct

SEQ ID NO: 521 - DNA, 20 bp, homo sapiens
gcactgtggttgagaattct

SEQ ID NO: 522 - DNA, 20 bp, homo sapiens
ttcacacatacaatgcactg

SEQ ID NO: 523 - DNA, 20 bp, homo sapiens
tatgtgtgaattacgttgtg

SEQ ID NO: 524 - DNA, 20 bp, homo sapiens
gacacattctgtttgttgaa

SEQ ID NO: 525 - DNA, 20 bp, homo sapiens
ggacacattctgtttgttga

SEQ ID NO: 526 - DNA, 20 bp, homo sapiens
aacagaatgtgtccttaaac

SEQ ID NO: 527 - DNA, 20 bp, homo sapiens
ctgaagattcaaccggttta

SEQ ID NO: 528 - DNA, 20 bp, homo sapiens
ttcatatctgaagattcaac

SEQ ID NO: 529 - DNA, 20 bp, homo sapiens
tgtatcttctgattcaactt

SEQ ID NO: 530 - DNA, 20 bp, homo sapiens
cctctttgacaaacttaaga

SEQ ID NO: 531 - DNA, 20 bp, homo sapiens
ccttcttaagtttgtcaaag

SEQ ID NO: 532 - DNA, 20 bp, homo sapiens
acctgatgctttaactttgc

SEQ ID NO: 533 - DNA, 20 bp, homo sapiens
gccagcaaagttaaagcatc

SEQ ID NO: 534 - DNA, 20 bp, homo sapiens
actttgctggccccagccgc

SEQ ID NO: 535 - DNA, 20 bp, homo sapiens
gattgtgtctccagcggctg

SEQ ID NO: 536 - DNA, 20 bp, homo sapiens
tgattgtgtctccagcggct

SEQ ID NO: 537 - DNA, 20 bp, homo sapiens
atgattgtgtctccagcggc

SEQ ID NO: 538 - DNA, 20 bp, homo sapiens
agatatgattgtgtctccag

SEQ ID NO: 539 - DNA, 20 bp, homo sapiens
acaatcatatctttagattt

SEQ ID NO: 540 - DNA, 20 bp, homo sapiens
tctttagattttggcagcaa

SEQ ID NO: 541 - DNA, 20 bp, homo sapiens
gtcatcagtttctgtgtctg

SEQ ID NO: 542 - DNA, 20 bp, homo sapiens
aactgatgaccagcaacttg

SEQ ID NO: 543 - DNA, 20 bp, homo sapiens
atggtacttcctcaagttgc

SEQ ID NO: 544 - DNA, 20 bp, homo sapiens
agcattacatcattatataa

SEQ ID NO: 545 - DNA, 20 bp, homo sapiens
gtaatttttcgttgggtgag

SEQ ID NO: 546 - DNA, 20 bp, homo sapiens
tgtaatttttcgttgggtga

SEQ ID NO: 547 - DNA, 20 bp, homo sapiens
ctgtaatttttcgttgggtg

SEQ ID NO: 548 - DNA, 20 bp, homo sapiens
atattctgtaatttttcgtt

SEQ ID NO: 549 - DNA, 20 bp, homo sapiens
tatattctgtaatttttcgt

SEQ ID NO: 550 - DNA, 20 bp, homo sapiens
aaaattacagaatataaatt

SEQ ID NO: 551 - DNA, 20 bp, homo sapiens
ggcgtttcagcggtgggtaa

SEQ ID NO: 552 - DNA, 20 bp, homo sapiens
ggctttggcgtttcagcggt

SEQ ID NO: 553 - DNA, 20 bp, homo sapiens
tggctttggcgtttcagcgg

SEQ ID NO: 554 - DNA, 20 bp, homo sapiens
aagtggctttggcgtttcag

SEQ ID NO: 555 - DNA, 20 bp, homo sapiens
gcactacttcgaagtggctt

SEQ ID NO: 556 - DNA, 20 bp, homo sapiens
gggtcagcactacttcgaag

SEQ ID NO: 557 - DNA, 20 bp, homo sapiens
caacttcttgattgagtgca

SEQ ID NO: 558 - DNA, 20 bp, homo sapiens
gcaacttcttgattgagtgc

SEQ ID NO: 559 - DNA, 20 bp, homo sapiens
agaaccaaatccagagtcac

SEQ ID NO: 560 - DNA, 20 bp, homo sapiens
agttccagtgactctggatt

SEQ ID NO: 561 - DNA, 20 bp, homo sapiens
aaagaaagttccagtgactc

SEQ ID NO: 562 - DNA, 20 bp, homo sapiens
ttttaccatgccccagattc

SEQ ID NO: 563 - DNA, 20 bp, homo sapiens
ctgatcctgaatctggggca

SEQ ID NO: 564 - DNA, 20 bp, homo sapiens
ggtgtctgatcctgaatctg

SEQ ID NO: 565 - DNA, 20 bp, homo sapiens
aggtgtctgatcctgaatct

SEQ ID NO: 566 - DNA, 20 bp, homo sapiens
taggtgtctgatcctgaatc

SEQ ID NO: 567 - DNA, 20 bp, homo sapiens
cagacacctagtccttccga

SEQ ID NO: 568 - DNA, 20 bp, homo sapiens
gtgcttccatcggaaggact

SEQ ID NO: 569 - DNA, 20 bp, homo sapiens
tgtctagtgcttccatcgga

SEQ ID NO: 570 - DNA, 20 bp, homo sapiens
actttgtctagtgcttccat

SEQ ID NO: 571 - DNA, 20 bp, homo sapiens
cactagacaaagttcacctg

SEQ ID NO: 572 - DNA, 20 bp, homo sapiens
agacaaagttcacctgaggt

SEQ ID NO: 573 - DNA, 20 bp, homo sapiens
tatatcatgacacctacctc

SEQ ID NO: 574 - DNA, 20 bp, homo sapiens
caatattcactgggactatt

SEQ ID NO: 575 - DNA, 20 bp, homo sapiens
acataaaaacaatattcact

SEQ ID NO: 576 - DNA, 20 bp, homo sapiens
cacataaaaacaatattcac

SEQ ID NO: 577 - DNA, 20 bp, homo sapiens
cagtgaatattgtttttatg

SEQ ID NO: 578 - DNA, 20 bp, homo sapiens
tttttatgtggatagtgata

SEQ ID NO: 579 - DNA, 20 bp, homo sapiens
tatggtcaatgaattcaagt

SEQ ID NO: 580 - DNA, 20 bp, homo sapiens
caatgaattcaagttggaat

SEQ ID NO: 581 - DNA, 20 bp, homo sapiens
aaagaacccattttctactc

SEQ ID NO: 582 - DNA, 20 bp, homo sapiens
catatacctgagtagaaaat

SEQ ID NO: 583 - DNA, 20 bp, homo sapiens
tcatatacctgagtagaaaa

SEQ ID NO: 584 - DNA, 20 bp, homo sapiens
aaaggacacagatttagact

SEQ ID NO: 585 - DNA, 20 bp, homo sapiens
gttagctccctatatcccaa

SEQ ID NO: 586 - DNA, 20 bp, homo sapiens
tcatcatccattgggatata

SEQ ID NO: 587 - DNA, 20 bp, homo sapiens
gtcatcatccattgggatat

SEQ ID NO: 588 - DNA, 20 bp, homo sapiens
actggaagtcatcatccatt

SEQ ID NO: 589 - DNA, 20 bp, homo sapiens
aactggaagtcatcatccat

SEQ ID NO: 590 - DNA, 20 bp, homo sapiens
actgatcgaaggaacgtaac

SEQ ID NO: 591 - DNA, 20 bp, homo sapiens
taatggtgacaactgatcga

SEQ ID NO: 592 - DNA, 20 bp, homo sapiens
cttgcggaactgctttctaa

SEQ ID NO: 593 - DNA, 20 bp, homo sapiens
acttgcgctttcagggcttg

SEQ ID NO: 594 - DNA, 20 bp, homo sapiens
tttgaggacttgcgctttca

SEQ ID NO: 595 - DNA, 20 bp, homo sapiens
ctttgaggacttgcgctttc

SEQ ID NO: 596 - DNA, 20 bp, homo sapiens
aatactgtaactgtgctttg

SEQ ID NO: 597 - DNA, 20 bp, homo sapiens
gttcttgtatttgagtctgc

SEQ ID NO: 598 - DNA, 20 bp, homo sapiens
gtagtggtggcattagcagt

SEQ ID NO: 599 - DNA, 20 bp, homo sapiens
agtggtggcagtggtagtgg

SEQ ID NO: 600 - DNA, 20 bp, homo sapiens
atcagtggtggcagtggtag

SEQ ID NO: 601 - DNA, 20 bp, homo sapiens
taattcatcagtggtggcag

SEQ ID NO: 602 - DNA, 20 bp, homo sapiens
tgtttttaattcatcagtgg

SEQ ID NO: 603 - DNA, 20 bp, homo sapiens
cactgtttttaattcatcag

SEQ ID NO: 604 - DNA, 20 bp, homo sapiens
aacagtgacaaaagaccgta

SEQ ID NO: 605 - DNA, 20 bp, homo sapiens
atattttaatgtcttccata

SEQ ID NO: 606 - DNA, 20 bp, homo sapiens
ttatgtatgtgggtaggaga

SEQ ID NO: 607 - DNA, 20 bp, homo sapiens
gtttctttatgtatgtgggt

SEQ ID NO: 608 - DNA, 20 bp, homo sapiens
agtagtttctttatgtatgt

SEQ ID NO: 609 - DNA, 20 bp, homo sapiens
tagtagtttctttatgtatg

SEQ ID NO: 610 - DNA, 20 bp, homo sapiens
atctctatatggtgatgatg

SEQ ID NO: 611 - DNA, 20 bp, homo sapiens
cgactttgagtatctctata

SEQ ID NO: 612 - DNA, 20 bp, homo sapiens
catatagagatactcaaagt

SEQ ID NO: 613 - DNA, 20 bp, homo sapiens
acagcctcaccaaacagagc

SEQ ID NO: 614 - DNA, 20 bp, homo sapiens
ttttcctgctctgtttggtg

SEQ ID NO: 615 - DNA, 20 bp, homo sapiens
tcaccaaacagagcaggaaa

SEQ ID NO: 616 - DNA, 20 bp, homo sapiens
actccttttcctgctctgtt

SEQ ID NO: 617 - DNA, 20 bp, homo sapiens
gataacacgttagggcttct

SEQ ID NO: 618 - DNA, 20 bp, homo sapiens
aagcgacagataacacgtta

SEQ ID NO: 619 - DNA, 20 bp, homo sapiens
aaagcgacagataacacgtt

SEQ ID NO: 620 - DNA, 20 bp, homo sapiens
tatctgtcgctttgagtcaa

SEQ ID NO: 621 - DNA, 20 bp, homo sapiens
tttcagaactacagttcctg

SEQ ID NO: 622 - DNA, 20 bp, homo sapiens
tttggatttagttcttcctc

SEQ ID NO: 623 - DNA, 20 bp, homo sapiens
ttctgcaaagctagtatctt

SEQ ID NO: 624 - DNA, 20 bp, homo sapiens
tgctcagagaaagcgaaaaa

SEQ ID NO: 625 - DNA, 20 bp, homo sapiens
aagcgaaaaatggaacatga

SEQ ID NO: 626 - DNA, 20 bp, homo sapiens
gtagtagctgcatgatcgtc

SEQ ID NO: 627 - DNA, 20 bp, homo sapiens
cagctactacatcactttct

SEQ ID NO: 628 - DNA, 20 bp, homo sapiens
ctttcttggaaacgtgtaaa

SEQ ID NO: 629 - DNA, 20 bp, homo sapiens
acaattattttaataccctc

SEQ ID NO: 630 - DNA, 20 bp, homo sapiens
aaaagaataaactaaccaga

SEQ ID NO: 631 - DNA, 20 bp, homo sapiens
aaaaagaataaactaaccag

SEQ ID NO: 632 - DNA, 20 bp, homo sapiens
agatttagcatgtagactgc

SEQ ID NO: 633 - DNA, 20 bp, homo sapiens
gatttagcatgtagactgct

SEQ ID NO: 634 - DNA, 20 bp, homo sapiens
atttagcatgtagactgctg

SEQ ID NO: 635 - DNA, 20 bp, homo sapiens
tagactgctggggcaatcaa

SEQ ID NO: 636 - DNA, 20 bp, homo sapiens
gggcaatcaatggatgaaag

SEQ ID NO: 637 - DNA, 20 bp, homo sapiens
caatcataactggtcagctg

SEQ ID NO: 638 - DNA, 20 bp, homo sapiens
attaacttcacaatcataac

SEQ ID NO: 639 - DNA, 20 bp, homo sapiens
gaagttaatgctcctataca

SEQ ID NO: 640 - DNA, 20 bp, homo sapiens
aggtttctgctgccttgtat

SEQ ID NO: 641 - DNA, 20 bp, homo sapiens
aggcagcagaaacctactgc

SEQ ID NO: 642 - DNA, 20 bp, homo sapiens
ggcagcagaaacctactgca

SEQ ID NO: 643 - DNA, 20 bp, homo sapiens
gtaattcttcaccctgcagt

SEQ ID NO: 644 - DNA, 20 bp, homo sapiens
tgaagaattactcagagctt

SEQ ID NO: 645 - DNA, 20 bp, homo sapiens
agcgacaatgacagctgaca

SEQ ID NO: 646 - DNA, 20 bp, homo sapiens
cagctgacaaggagaagaaa

SEQ ID NO: 647 - DNA, 20 bp, homo sapiens
ttctccacttaggagtagct

SEQ ID NO: 648 - DNA, 20 bp, homo sapiens
cacttaggagtagctcggag

SEQ ID NO: 649 - DNA, 20 bp, homo sapiens
ttaggagtagctcggagagg

SEQ ID NO: 650 - DNA, 20 bp, homo sapiens
gagtagctcggagaggagga

SEQ ID NO: 651 - DNA, 20 bp, homo sapiens
agaggaggaaggagaagtcc

SEQ ID NO: 652 - DNA, 20 bp, homo sapiens
gaggaggaaggagaagtccc

SEQ ID NO: 653 - DNA, 20 bp, homo sapiens
agaagtcccgggatgctgcg

SEQ ID NO: 654 - DNA, 20 bp, homo sapiens
cccgggatgctgcgcggtgc

SEQ ID NO: 655 - DNA, 20 bp, homo sapiens
ccggcaccgcgcagcatccc

SEQ ID NO: 656 - DNA, 20 bp, homo sapiens
gccggcaccgcgcagcatcc

SEQ ID NO: 657 - DNA, 20 bp, homo sapiens
gggatgctgcgcggtgccgg

SEQ ID NO: 658 - DNA, 20 bp, homo sapiens
tgcgcggtgccggcggagca

SEQ ID NO: 659 - DNA, 20 bp, homo sapiens
gtgccggcggagcaaggaga

SEQ ID NO: 660 - DNA, 20 bp, homo sapiens
ccggcggagcaaggagacgg

SEQ ID NO: 661 - DNA, 20 bp, homo sapiens
cctccgtctccttgctccgc

SEQ ID NO: 662 - DNA, 20 bp, homo sapiens
gacggaggtgttctatgagc

SEQ ID NO: 663 - DNA, 20 bp, homo sapiens
gtggggcagaggcagctcat

SEQ ID NO: 664 - DNA, 20 bp, homo sapiens
tgtggggcagaggcagctca

SEQ ID NO: 665 - DNA, 20 bp, homo sapiens
gagctcacactgtggggcag

SEQ ID NO: 666 - DNA, 20 bp, homo sapiens
agatgggagctcacactgtg

SEQ ID NO: 667 - DNA, 20 bp, homo sapiens
cagatgggagctcacactgt

SEQ ID NO: 668 - DNA, 20 bp, homo sapiens
ccacagtgtgagctcccatc

SEQ ID NO: 669 - DNA, 20 bp, homo sapiens
ccagatgggagctcacactg

SEQ ID NO: 670 - DNA, 20 bp, homo sapiens
tgtgagctcccatctggaca

SEQ ID NO: 671 - DNA, 20 bp, homo sapiens
gatggaggccttgtccagat

SEQ ID NO: 672 - DNA, 20 bp, homo sapiens
tgatggaggccttgtccaga

SEQ ID NO: 673 - DNA, 20 bp, homo sapiens
caaggcctccatcatgcgac

SEQ ID NO: 674 - DNA, 20 bp, homo sapiens
gattgccagtcgcatgatgg

SEQ ID NO: 675 - DNA, 20 bp, homo sapiens
gctgattgccagtcgcatga

SEQ ID NO: 676 - DNA, 20 bp, homo sapiens
agaggagcttgtgtgttcgc

SEQ ID NO: 677 - DNA, 20 bp, homo sapiens
acacacaagctcctctcctc

SEQ ID NO: 678 - DNA, 20 bp, homo sapiens
caagctcctctcctcaggta

SEQ ID NO: 679 - DNA, 20 bp, homo sapiens
tgctggccttacctgaggag

SEQ ID NO: 680 - DNA, 20 bp, homo sapiens
gagcctgctggccttacctg

SEQ ID NO: 681 - DNA, 20 bp, homo sapiens
gactcgttttcagagcaaac

SEQ ID NO: 682 - DNA, 20 bp, homo sapiens
ctgctggtcagcttcggctt

SEQ ID NO: 683 - DNA, 20 bp, homo sapiens
agccgaagctgaccagcaga

SEQ ID NO: 684 - DNA, 20 bp, homo sapiens
gtccatctgctggtcagctt

SEQ ID NO: 685 - DNA, 20 bp, homo sapiens
ggtacaagttgtccatctgc

SEQ ID NO: 686 - DNA, 20 bp, homo sapiens
caacttgtacctgaaagcct

SEQ ID NO: 687 - DNA, 20 bp, homo sapiens
cttgtacctgaaagccttgg

SEQ ID NO: 688 - DNA, 20 bp, homo sapiens
ttgtacctgaaagccttgga

SEQ ID NO: 689 - DNA, 20 bp, homo sapiens
tgaaaccctccaaggctttc

SEQ ID NO: 690 - DNA, 20 bp, homo sapiens
cacggcaatgaaaccctcca

SEQ ID NO: 691 - DNA, 20 bp, homo sapiens
cttggagggtttcattgccg

SEQ ID NO: 692 - DNA, 20 bp, homo sapiens
attgccgtggtgacccaaga

SEQ ID NO: 693 - DNA, 20 bp, homo sapiens
gtcgccatcttgggtcacca

SEQ ID NO: 694 - DNA, 20 bp, homo sapiens
aaagatcatgtcgccatctt

SEQ ID NO: 695 - DNA, 20 bp, homo sapiens
gaaagatcatgtcgccatct

SEQ ID NO: 696 - DNA, 20 bp, homo sapiens
agaaaacatcagcaagttca

SEQ ID NO: 697 - DNA, 20 bp, homo sapiens
gaaaacatcagcaagttcat

SEQ ID NO: 698 - DNA, 20 bp, homo sapiens
caagttcatgggacttacac

SEQ ID NO: 699 - DNA, 20 bp, homo sapiens
ttgaaacaggtggagctaac

SEQ ID NO: 700 - DNA, 20 bp, homo sapiens
cactcatccctgcgaccatg

SEQ ID NO: 701 - DNA, 20 bp, homo sapiens
cgaatctcctcatggtcgca

SEQ ID NO: 702 - DNA, 20 bp, homo sapiens
acgaatctcctcatggtcgc

SEQ ID NO: 703 - DNA, 20 bp, homo sapiens
ggttctcacgaatctcctca

SEQ ID NO: 704 - DNA, 20 bp, homo sapiens
gagaacctgagtctcaaaaa

SEQ ID NO: 705 - DNA, 20 bp, homo sapiens
ggataccatttttgagactc

SEQ ID NO: 706 - DNA, 20 bp, homo sapiens
atccttccacatccaggctc

SEQ ID NO: 707 - DNA, 20 bp, homo sapiens
ccacatccaggctctggttt

SEQ ID NO: 708 - DNA, 20 bp, homo sapiens
cacatccaggctctggtttt

SEQ ID NO: 709 - DNA, 20 bp, homo sapiens
tttttcccaaaaccagagcc

SEQ ID NO: 710 - DNA, 20 bp, homo sapiens
gcaaagacatgtccacagag

SEQ ID NO: 711 - DNA, 20 bp, homo sapiens
caaagacatgtccacagagc

SEQ ID NO: 712 - DNA, 20 bp, homo sapiens
catgaagaagtcccgctctg

SEQ ID NO: 713 - DNA, 20 bp, homo sapiens
cagagcgggacttcttcatg

SEQ ID NO: 714 - DNA, 20 bp, homo sapiens
cttcatgaggatgaagtgca

SEQ ID NO: 715 - DNA, 20 bp, homo sapiens
aagtgcacggtcaccaacag

SEQ ID NO: 716 - DNA, 20 bp, homo sapiens
gttgacagtacggcctctgt

SEQ ID NO: 717 - DNA, 20 bp, homo sapiens
ctgacttgaggttgacagta

SEQ ID NO: 718 - DNA, 20 bp, homo sapiens
tcaacctcaagtcagccacc

SEQ ID NO: 719 - DNA, 20 bp, homo sapiens
cctcaagtcagccacctgga

SEQ ID NO: 720 - DNA, 20 bp, homo sapiens
ccttccaggtggctgacttg

SEQ ID NO: 721 - DNA, 20 bp, homo sapiens
aagtcagccacctggaaggt

SEQ ID NO: 722 - DNA, 20 bp, homo sapiens
agtcagccacctggaaggta

SEQ ID NO: 723 - DNA, 20 bp, homo sapiens
atgttgccctaccttccagg

SEQ ID NO: 724 - DNA, 20 bp, homo sapiens
ctgatgttgccctaccttcc

SEQ ID NO: 725 - DNA, 20 bp, homo sapiens
gtctcaggtcttgcactgca

SEQ ID NO: 726 - DNA, 20 bp, homo sapiens
tctcaggtcttgcactgcac

SEQ ID NO: 727 - DNA, 20 bp, homo sapiens
ggtcttgcactgcacgggcc

SEQ ID NO: 728 - DNA, 20 bp, homo sapiens
agttgttgtagactttcacc

SEQ ID NO: 729 - DNA, 20 bp, homo sapiens
cacacagactattgtgagga

SEQ ID NO: 730 - DNA, 20 bp, homo sapiens
cctcctcacaatagtctgtg

SEQ ID NO: 731 - DNA, 20 bp, homo sapiens
ccacacagactattgtgagg

SEQ ID NO: 732 - DNA, 20 bp, homo sapiens
tagccacacagactattgtg

SEQ ID NO: 733 - DNA, 20 bp, homo sapiens
caatagtctgtgtggctaca

SEQ ID NO: 734 - DNA, 20 bp, homo sapiens
atgatgaggcaggacagcag

SEQ ID NO: 735 - DNA, 20 bp, homo sapiens
gatgatgaggcaggacagca

SEQ ID NO: 736 - DNA, 20 bp, homo sapiens
tgatgatgaggcaggacagc

SEQ ID NO: 737 - DNA, 20 bp, homo sapiens
ttcacacatgatgatgaggc

SEQ ID NO: 738 - DNA, 20 bp, homo sapiens
ttggttcacacatgatgatg

SEQ ID NO: 739 - DNA, 20 bp, homo sapiens
atgtgggatgggtgctggat

SEQ ID NO: 740 - DNA, 20 bp, homo sapiens
aatccagcacccatcccaca

SEQ ID NO: 741 - DNA, 20 bp, homo sapiens
tgtccatgtgggatgggtgc

SEQ ID NO: 742 - DNA, 20 bp, homo sapiens
gggggatgtccatgtgggat

SEQ ID NO: 743 - DNA, 20 bp, homo sapiens
agggggatgtccatgtggga

SEQ ID NO: 744 - DNA, 20 bp, homo sapiens
atcccacatggacatccccc

SEQ ID NO: 745 - DNA, 20 bp, homo sapiens
atccagggggatgtccatgt

SEQ ID NO: 746 - DNA, 20 bp, homo sapiens
tatccagggggatgtccatg

SEQ ID NO: 747 - DNA, 20 bp, homo sapiens
ggaaggtcttgctatccagg

SEQ ID NO: 748 - DNA, 20 bp, homo sapiens
aggaaggtcttgctatccag

SEQ ID NO: 749 - DNA, 20 bp, homo sapiens
caggaaggtcttgctatcca

SEQ ID NO: 750 - DNA, 20 bp, homo sapiens
tcaggaaggtcttgctatcc

SEQ ID NO: 751 - DNA, 20 bp, homo sapiens
catgctgtggcggctcagga

SEQ ID NO: 752 - DNA, 20 bp, homo sapiens
cttcctgagccgccacagca

SEQ ID NO: 753 - DNA, 20 bp, homo sapiens
tgtccatgctgtggcggctc

SEQ ID NO: 754 - DNA, 20 bp, homo sapiens
acttcatgtccatgctgtgg

SEQ ID NO: 755 - DNA, 20 bp, homo sapiens
tgaacttcatgtccatgctg

SEQ ID NO: 756 - DNA, 20 bp, homo sapiens
agttcacctactgtgatgac

SEQ ID NO: 757 - DNA, 20 bp, homo sapiens
cacctactgtgatgacaggt

SEQ ID NO: 758 - DNA, 20 bp, homo sapiens
acctactgtgatgacaggta

SEQ ID NO: 759 - DNA, 20 bp, homo sapiens
cccctacctgtcatcacagt

SEQ ID NO: 760 - DNA, 20 bp, homo sapiens
ctcagaatcacagaactgat

SEQ ID NO: 761 - DNA, 20 bp, homo sapiens
actgattggttaccaccctg

SEQ ID NO: 762 - DNA, 20 bp, homo sapiens
taccaccctgaggagctgct

SEQ ID NO: 763 - DNA, 20 bp, homo sapiens
ggccaagcagctcctcaggg

SEQ ID NO: 764 - DNA, 20 bp, homo sapiens
agcggccaagcagctcctca

SEQ ID NO: 765 - DNA, 20 bp, homo sapiens
gagcggccaagcagctcctc

SEQ ID NO: 766 - DNA, 20 bp, homo sapiens
ggtagaattcataggctgag

SEQ ID NO: 767 - DNA, 20 bp, homo sapiens
tagcgcatggtagaattcat

SEQ ID NO: 768 - DNA, 20 bp, homo sapiens
tgttctcggagtctagcgca

SEQ ID NO: 769 - DNA, 20 bp, homo sapiens
gtgactcttggtcatgttct

SEQ ID NO: 770 - DNA, 20 bp, homo sapiens
ctcacagttctggtgactct

SEQ ID NO: 771 - DNA, 20 bp, homo sapiens
actcctggaactcacagttc

SEQ ID NO: 772 - DNA, 20 bp, homo sapiens
tcctcccctagtgtgcacca

SEQ ID NO: 773 - DNA, 20 bp, homo sapiens
cctcccctagtgtgcaccaa

SEQ ID NO: 774 - DNA, 20 bp, homo sapiens
ctgacccttggtgcacacta

SEQ ID NO: 775 - DNA, 20 bp, homo sapiens
cctagtgtgcaccaagggtc

SEQ ID NO: 776 - DNA, 20 bp, homo sapiens
cctgacccttggtgcacact

SEQ ID NO: 777 - DNA, 20 bp, homo sapiens
accaagggtcaggtagtaag

SEQ ID NO: 778 - DNA, 20 bp, homo sapiens
gccacttactacctgaccct

SEQ ID NO: 779 - DNA, 20 bp, homo sapiens
aggtagtaagtggccagtac

SEQ ID NO: 780 - DNA, 20 bp, homo sapiens
gctttgcgagcatccggtac

SEQ ID NO: 781 - DNA, 20 bp, homo sapiens
taccggatgctcgcaaagca

SEQ ID NO: 782 - DNA, 20 bp, homo sapiens
accggatgctcgcaaagcat

SEQ ID NO: 783 - DNA, 20 bp, homo sapiens
ccggatgctcgcaaagcatg

SEQ ID NO: 784 - DNA, 20 bp, homo sapiens
ccccatgctttgcgagcatc

SEQ ID NO: 785 - DNA, 20 bp, homo sapiens
cggatgctcgcaaagcatgg

SEQ ID NO: 786 - DNA, 20 bp, homo sapiens
caaagcatgggggctacgtg

SEQ ID NO: 787 - DNA, 20 bp, homo sapiens
gcatgggggctacgtgtggc

SEQ ID NO: 788 - DNA, 20 bp, homo sapiens
ctacgtgtggctggagaccc

SEQ ID NO: 789 - DNA, 20 bp, homo sapiens
tacgtgtggctggagaccca

SEQ ID NO: 790 - DNA, 20 bp, homo sapiens
acgtgtggctggagacccag

SEQ ID NO: 791 - DNA, 20 bp, homo sapiens
gtggctggagacccagggga

SEQ ID NO: 792 - DNA, 20 bp, homo sapiens
gttgtagatgaccgtcccct

SEQ ID NO: 793 - DNA, 20 bp, homo sapiens
ggttgtagatgaccgtcccc

SEQ ID NO: 794 - DNA, 20 bp, homo sapiens
actggggctgcaggttgcga

SEQ ID NO: 795 - DNA, 20 bp, homo sapiens
cactggggctgcaggttgcg

SEQ ID NO: 796 - DNA, 20 bp, homo sapiens
acatgatgcactggggctgc

SEQ ID NO: 797 - DNA, 20 bp, homo sapiens
ttgacacacatgatgcactg

SEQ ID NO: 798 - DNA, 20 bp, homo sapiens
gttgacacacatgatgcact

SEQ ID NO: 799 - DNA, 20 bp, homo sapiens
agttgacacacatgatgcac

SEQ ID NO: 800 - DNA, 20 bp, homo sapiens
tgtgtgtcaactacgtcctg

SEQ ID NO: 801 - DNA, 20 bp, homo sapiens
agccctcacatgcttacctc

SEQ ID NO: 802 - DNA, 20 bp, homo sapiens
tgagattgagaagaatgacg

SEQ ID NO: 803 - DNA, 20 bp, homo sapiens
gaatgacgtggtgttctcca

SEQ ID NO: 804 - DNA, 20 bp, homo sapiens
cagggattcagtctggtcca

SEQ ID NO: 805 - DNA, 20 bp, homo sapiens
gcttgaacagggattcagtc

SEQ ID NO: 806 - DNA, 20 bp, homo sapiens
catcaggtggggcttgaaca

SEQ ID NO: 807 - DNA, 20 bp, homo sapiens
cctgttcaagccccacctga

SEQ ID NO: 808 - DNA, 20 bp, homo sapiens
ccatcaggtggggcttgaac

SEQ ID NO: 809 - DNA, 20 bp, homo sapiens
ctgttcatggccatcaggtg

SEQ ID NO: 810 - DNA, 20 bp, homo sapiens
gctgttcatggccatcaggt

SEQ ID NO: 811 - DNA, 20 bp, homo sapiens
tgctgttcatggccatcagg

SEQ ID NO: 812 - DNA, 20 bp, homo sapiens
agatgctgttcatggccatc

SEQ ID NO: 813 - DNA, 20 bp, homo sapiens
gctatcaaagatgctgttca

SEQ ID NO: 814 - DNA, 20 bp, homo sapiens
aacagcatctttgatagcag

SEQ ID NO: 815 - DNA, 20 bp, homo sapiens
catctttgatagcagtggca

SEQ ID NO: 816 - DNA, 20 bp, homo sapiens
atctttgatagcagtggcaa

SEQ ID NO: 817 - DNA, 20 bp, homo sapiens
tctttgatagcagtggcaag

SEQ ID NO: 818 - DNA, 20 bp, homo sapiens
ctttgatagcagtggcaagg

SEQ ID NO: 819 - DNA, 20 bp, homo sapiens
cttcctattcaccaagctaa

SEQ ID NO: 820 - DNA, 20 bp, homo sapiens
cctattcaccaagctaaagg

SEQ ID NO: 821 - DNA, 20 bp, homo sapiens
cctcctttagcttggtgaat

SEQ ID NO: 822 - DNA, 20 bp, homo sapiens
ctcgggctcctcctttagct

SEQ ID NO: 823 - DNA, 20 bp, homo sapiens
caagctaaaggaggagcccg

SEQ ID NO: 824 - DNA, 20 bp, homo sapiens
aaaggaggagcccgaggagc

SEQ ID NO: 825 - DNA, 20 bp, homo sapiens
gcccgaggagctggcccagc

SEQ ID NO: 826 - DNA, 20 bp, homo sapiens
gccagctgggccagctcctc

SEQ ID NO: 827 - DNA, 20 bp, homo sapiens
agccagctgggccagctcct

SEQ ID NO: 828 - DNA, 20 bp, homo sapiens
gcccagctggctcccacccc

SEQ ID NO: 829 - DNA, 20 bp, homo sapiens
tcctggggtgggagccagct

SEQ ID NO: 830 - DNA, 20 bp, homo sapiens
ctcctggggtgggagccagc

SEQ ID NO: 831 - DNA, 20 bp, homo sapiens
atgatggcgtctcctggggt

SEQ ID NO: 832 - DNA, 20 bp, homo sapiens
gatgatggcgtctcctgggg

SEQ ID NO: 833 - DNA, 20 bp, homo sapiens
agagatgatggcgtctcctg

SEQ ID NO: 834 - DNA, 20 bp, homo sapiens
gagagatgatggcgtctcct

SEQ ID NO: 835 - DNA, 20 bp, homo sapiens
agagagatgatggcgtctcc

SEQ ID NO: 836 - DNA, 20 bp, homo sapiens
aggagacgccatcatctctc

SEQ ID NO: 837 - DNA, 20 bp, homo sapiens
gccatcatctctctggattt

SEQ ID NO: 838 - DNA, 20 bp, homo sapiens
accgaaatccagagagatga

SEQ ID NO: 839 - DNA, 20 bp, homo sapiens
atcatctctctggatttcgg

SEQ ID NO: 840 - DNA, 20 bp, homo sapiens
tcatctctctggatttcggt

SEQ ID NO: 841 - DNA, 20 bp, homo sapiens
ctcgaagttctgattccctg

SEQ ID NO: 842 - DNA, 20 bp, homo sapiens
cacagggaatcagaacttcg

SEQ ID NO: 843 - DNA, 20 bp, homo sapiens
ttcgaggagtcctcagccta

SEQ ID NO: 844 - DNA, 20 bp, homo sapiens
ggagtcctcagcctatggca

SEQ ID NO: 845 - DNA, 20 bp, homo sapiens
gatggccttgccataggctg

SEQ ID NO: 846 - DNA, 20 bp, homo sapiens
gggcaggatggccttgccat

SEQ ID NO: 847 - DNA, 20 bp, homo sapiens
tggctggctcgggggcagga

SEQ ID NO: 848 - DNA, 20 bp, homo sapiens
tcctgcccccgagccagcca

SEQ ID NO: 849 - DNA, 20 bp, homo sapiens
cctgcccccgagccagccat

SEQ ID NO: 850 - DNA, 20 bp, homo sapiens
cccatggctggctcgggggc

SEQ ID NO: 851 - DNA, 20 bp, homo sapiens
gtggcccatggctggctcgg

SEQ ID NO: 852 - DNA, 20 bp, homo sapiens
cgtggcccatggctggctcg

SEQ ID NO: 853 - DNA, 20 bp, homo sapiens
cccgagccagccatgggcca

SEQ ID NO: 854 - DNA, 20 bp, homo sapiens
ccgtggcccatggctggctc

SEQ ID NO: 855 - DNA, 20 bp, homo sapiens
tccgtggcccatggctggct

SEQ ID NO: 856 - DNA, 20 bp, homo sapiens
tcaactccgtggcccatggc

SEQ ID NO: 857 - DNA, 20 bp, homo sapiens
agccatgggccacggagttg

SEQ ID NO: 858 - DNA, 20 bp, homo sapiens
ctcctcaactccgtggccca

SEQ ID NO: 859 - DNA, 20 bp, homo sapiens
gctgtggctcctcaactccg

SEQ ID NO: 860 - DNA, 20 bp, homo sapiens
gagccacagcacccagagcg

SEQ ID NO: 861 - DNA, 20 bp, homo sapiens
cagcctcgctctgggtgctg

SEQ ID NO: 862 - DNA, 20 bp, homo sapiens
cacagcacccagagcgaggc

SEQ ID NO: 863 - DNA, 20 bp, homo sapiens
acagcacccagagcgaggct

SEQ ID NO: 864 - DNA, 20 bp, homo sapiens
caggctcccagcctcgctct

SEQ ID NO: 865 - DNA, 20 bp, homo sapiens
gcaggctcccagcctcgctc

SEQ ID NO: 866 - DNA, 20 bp, homo sapiens
ggggcacggtgaaggcaggc

SEQ ID NO: 867 - DNA, 20 bp, homo sapiens
gcctgccttcaccgtgcccc

SEQ ID NO: 868 - DNA, 20 bp, homo sapiens
gcctggggcacggtgaaggc

SEQ ID NO: 869 - DNA, 20 bp, homo sapiens
agctgcctggggcacggtga

SEQ ID NO: 870 - DNA, 20 bp, homo sapiens
cggggcagctgcctggggca

SEQ ID NO: 871 - DNA, 20 bp, homo sapiens
cgtgccccaggcagctgccc

SEQ ID NO: 872 - DNA, 20 bp, homo sapiens
gtgccccaggcagctgcccc

SEQ ID NO: 873 - DNA, 20 bp, homo sapiens
ctgcccggggcagctgcctg

SEQ ID NO: 874 - DNA, 20 bp, homo sapiens
gctgcccggggcagctgcct

SEQ ID NO: 875 - DNA, 20 bp, homo sapiens
tgctgcccggggcagctgcc

SEQ ID NO: 876 - DNA, 20 bp, homo sapiens
actgggggtggtgctgcccg

SEQ ID NO: 877 - DNA, 20 bp, homo sapiens
cactgggggtggtgctgccc

SEQ ID NO: 878 - DNA, 20 bp, homo sapiens
gcactgggggtggtgctgcc

SEQ ID NO: 879 - DNA, 20 bp, homo sapiens
gctgctggtggcactggggg

SEQ ID NO: 880 - DNA, 20 bp, homo sapiens
gctgctgctggtggcactgg

SEQ ID NO: 881 - DNA, 20 bp, homo sapiens
tgctgctgctggtggcactg

SEQ ID NO: 882 - DNA, 20 bp, homo sapiens
ctgctgctgctggtggcact

SEQ ID NO: 883 - DNA, 20 bp, homo sapiens
gctgctgctgctggtggcac

SEQ ID NO: 884 - DNA, 20 bp, homo sapiens
gcagctgctgctgctgctgg

SEQ ID NO: 885 - DNA, 20 bp, homo sapiens
cagcagcagcagctgctcca

SEQ ID NO: 886 - DNA, 20 bp, homo sapiens
tcttcagggctattgggcta

SEQ ID NO: 887 - DNA, 20 bp, homo sapiens
gtcttcagggctattgggct

SEQ ID NO: 888 - DNA, 20 bp, homo sapiens
taatagtcttcagggctatt

SEQ ID NO: 889 - DNA, 20 bp, homo sapiens
gtaatagtcttcagggctat

SEQ ID NO: 890 - DNA, 20 bp, homo sapiens
aagatgtgtaatagtcttca

SEQ ID NO: 891 - DNA, 20 bp, homo sapiens
aaagatgtgtaatagtcttc

SEQ ID NO: 892 - DNA, 20 bp, homo sapiens
tgaagactattacacatctt

SEQ ID NO: 893 - DNA, 20 bp, homo sapiens
tctcaatcacttcaatcttc

SEQ ID NO: 894 - DNA, 20 bp, homo sapiens
gattgagaagctcttcgcca

SEQ ID NO: 895 - DNA, 20 bp, homo sapiens
gctcttcgccatggacacag

SEQ ID NO: 896 - DNA, 20 bp, homo sapiens
cgccatggacacagaggcca

SEQ ID NO: 897 - DNA, 20 bp, homo sapiens
gtccttggcctctgtgtcca

SEQ ID NO: 898 - DNA, 20 bp, homo sapiens
ctgggtactgcattggtcct

SEQ ID NO: 899 - DNA, 20 bp, homo sapiens
caaggaccaatgcagtaccc

SEQ ID NO: 900 - DNA, 20 bp, homo sapiens
catctacctgggtactgcat

SEQ ID NO: 901 - DNA, 20 bp, homo sapiens
agctcattgaaatccgtctg

SEQ ID NO: 902 - DNA, 20 bp, homo sapiens
tcagacggatttcaatgagc

SEQ ID NO: 903 - DNA, 20 bp, homo sapiens
ggatttcaatgagctggact

SEQ ID NO: 904 - DNA, 20 bp, homo sapiens
tgagctggacttggagacac

SEQ ID NO: 905 - DNA, 20 bp, homo sapiens
actggcaccctatatcccca

SEQ ID NO: 906 - DNA, 20 bp, homo sapiens
gcaccctatatccccatgga

SEQ ID NO: 907 - DNA, 20 bp, homo sapiens
caccctatatccccatggac

SEQ ID NO: 908 - DNA, 20 bp, homo sapiens
accctatatccccatggacg

SEQ ID NO: 909 - DNA, 20 bp, homo sapiens
tccccgtccatggggatata

SEQ ID NO: 910 - DNA, 20 bp, homo sapiens
ttccccgtccatggggatat

SEQ ID NO: 911 - DNA, 20 bp, homo sapiens
ggaagtcttccccgtccatg

SEQ ID NO: 912 - DNA, 20 bp, homo sapiens
tggaagtcttccccgtccat

SEQ ID NO: 913 - DNA, 20 bp, homo sapiens
ctggaagtcttccccgtcca

SEQ ID NO: 914 - DNA, 20 bp, homo sapiens
cggggcagatggggcttagc

SEQ ID NO: 915 - DNA, 20 bp, homo sapiens
gctaagccccatctgccccg

SEQ ID NO: 916 - DNA, 20 bp, homo sapiens
gccccatctgccccgaggag

SEQ ID NO: 917 - DNA, 20 bp, homo sapiens
gccgctcctcggggcagatg

SEQ ID NO: 918 - DNA, 20 bp, homo sapiens
agccgctcctcggggcagat

SEQ ID NO: 919 - DNA, 20 bp, homo sapiens
gagccgctcctcggggcaga

SEQ ID NO: 920 - DNA, 20 bp, homo sapiens
ctgccccgaggagcggctct

SEQ ID NO: 921 - DNA, 20 bp, homo sapiens
ccccgaggagcggctcttgg

SEQ ID NO: 922 - DNA, 20 bp, homo sapiens
ccgccaagagccgctcctcg

SEQ ID NO: 923 - DNA, 20 bp, homo sapiens
tccgccaagagccgctcctc

SEQ ID NO: 924 - DNA, 20 bp, homo sapiens
ctccgccaagagccgctcct

SEQ ID NO: 925 - DNA, 20 bp, homo sapiens
agtgctggggggtggactgt

SEQ ID NO: 926 - DNA, 20 bp, homo sapiens
cagtgctggggggtggactg

SEQ ID NO: 927 - DNA, 20 bp, homo sapiens
actgaagcagtgctgggggg

SEQ ID NO: 928 - DNA, 20 bp, homo sapiens
ggcactgaagcagtgctggg

SEQ ID NO: 929 - DNA, 20 bp, homo sapiens
tggcactgaagcagtgctgg

SEQ ID NO: 930 - DNA, 20 bp, homo sapiens
atggcactgaagcagtgctg

SEQ ID NO: 931 - DNA, 20 bp, homo sapiens
catggcactgaagcagtgct

SEQ ID NO: 932 - DNA, 20 bp, homo sapiens
tcatggcactgaagcagtgc

SEQ ID NO: 933 - DNA, 20 bp, homo sapiens
tggctggaagatgtttgtca

SEQ ID NO: 934 - DNA, 20 bp, homo sapiens
gacaaacatcttccagccac

SEQ ID NO: 935 - DNA, 20 bp, homo sapiens
gggctacaggggccagtggc

SEQ ID NO: 936 - DNA, 20 bp, homo sapiens
tgcggggctacaggggccag

SEQ ID NO: 937 - DNA, 20 bp, homo sapiens
gggactgtgcggggctacag

SEQ ID NO: 938 - DNA, 20 bp, homo sapiens
agggactgtgcggggctaca

SEQ ID NO: 939 - DNA, 20 bp, homo sapiens
aagggactgtgcggggctac

SEQ ID NO: 940 - DNA, 20 bp, homo sapiens
caggaggaagggactgtgcg

SEQ ID NO: 941 - DNA, 20 bp, homo sapiens
cccgcacagtcccttcctcc

SEQ ID NO: 942 - DNA, 20 bp, homo sapiens
ccaggaggaagggactgtgc

SEQ ID NO: 943 - DNA, 20 bp, homo sapiens
tccaggaggaagggactgtg

SEQ ID NO: 944 - DNA, 20 bp, homo sapiens
tgaaacttgtccaggaggaa

SEQ ID NO: 945 - DNA, 20 bp, homo sapiens
ctgaaacttgtccaggagga

SEQ ID NO: 946 - DNA, 20 bp, homo sapiens
gctgctgaaacttgtccagg

SEQ ID NO: 947 - DNA, 20 bp, homo sapiens
gctgctgctgaaacttgtcc

SEQ ID NO: 948 - DNA, 20 bp, homo sapiens
ggacaagtttcagcagcagc

SEQ ID NO: 949 - DNA, 20 bp, homo sapiens
agaagacagagcccgagcac

SEQ ID NO: 950 - DNA, 20 bp, homo sapiens
gaggacatgggccggtgctc

SEQ ID NO: 951 - DNA, 20 bp, homo sapiens
ggaggacatgggccggtgct

SEQ ID NO: 952 - DNA, 20 bp, homo sapiens
agaagatggaggacatgggc

SEQ ID NO: 953 - DNA, 20 bp, homo sapiens
tcaaagaagatggaggacat

SEQ ID NO: 954 - DNA, 20 bp, homo sapiens
atcaaagaagatggaggaca

SEQ ID NO: 955 - DNA, 20 bp, homo sapiens
tcctccatcttctttgatgc

SEQ ID NO: 956 - DNA, 20 bp, homo sapiens
tccggcatcaaagaagatgg

SEQ ID NO: 957 - DNA, 20 bp, homo sapiens
gcttccggcatcaaagaaga

SEQ ID NO: 958 - DNA, 20 bp, homo sapiens
tggcagggatgctttgcttc

SEQ ID NO: 959 - DNA, 20 bp, homo sapiens
gcatccctgccaccgtgctg

SEQ ID NO: 960 - DNA, 20 bp, homo sapiens
ctggccacagcacggtggca

SEQ ID NO: 961 - DNA, 20 bp, homo sapiens
cctgccaccgtgctgtggcc

SEQ ID NO: 962 - DNA, 20 bp, homo sapiens
cctggccacagcacggtggc

SEQ ID NO: 963 - DNA, 20 bp, homo sapiens
ctggcctggccacagcacgg

SEQ ID NO: 964 - DNA, 20 bp, homo sapiens
gtgctggcctggccacagca

SEQ ID NO: 965 - DNA, 20 bp, homo sapiens
aagagagaggggtgctggcc

SEQ ID NO: 966 - DNA, 20 bp, homo sapiens
catggaagagagaggggtgc

SEQ ID NO: 967 - DNA, 20 bp, homo sapiens
cagcacccctctctcttcca

SEQ ID NO: 968 - DNA, 20 bp, homo sapiens
agcacccctctctcttccat

SEQ ID NO: 969 - DNA, 20 bp, homo sapiens
gcacccctctctcttccatg

SEQ ID NO: 970 - DNA, 20 bp, homo sapiens
cacccctctctcttccatgg

SEQ ID NO: 971 - DNA, 20 bp, homo sapiens
acccctctctcttccatggg

SEQ ID NO: 972 - DNA, 20 bp, homo sapiens
gccccccatggaagagagag

SEQ ID NO: 973 - DNA, 20 bp, homo sapiens
tgccccccatggaagagaga

SEQ ID NO: 974 - DNA, 20 bp, homo sapiens
ctgccccccatggaagagag

SEQ ID NO: 975 - DNA, 20 bp, homo sapiens
ggtattggatctgcccccca

SEQ ID NO: 976 - DNA, 20 bp, homo sapiens
ggggcagatccaatacccag

SEQ ID NO: 977 - DNA, 20 bp, homo sapiens
atctgggggccactgggtat

SEQ ID NO: 978 - DNA, 20 bp, homo sapiens
tggtggatctgggggccact

SEQ ID NO: 979 - DNA, 20 bp, homo sapiens
atggtggatctgggggccac

SEQ ID NO: 980 - DNA, 20 bp, homo sapiens
aaatgtaatggtggatctgg

SEQ ID NO: 981 - DNA, 20 bp, homo sapiens
aaaatgtaatggtggatctg

SEQ ID NO: 982 - DNA, 20 bp, homo sapiens
caaaatgtaatggtggatct

SEQ ID NO: 983 - DNA, 20 bp, homo sapiens
ccagatccaccattacattt

SEQ ID NO: 984 - DNA, 20 bp, homo sapiens
ccaaaatgtaatggtggatc

SEQ ID NO: 985 - DNA, 20 bp, homo sapiens
cagatccaccattacatttt

SEQ ID NO: 986 - DNA, 20 bp, homo sapiens
gtgggcccaaaatgtaatgg

SEQ ID NO: 987 - DNA, 20 bp, homo sapiens
tttgtgggcccaaaatgtaa

SEQ ID NO: 988 - DNA, 20 bp, homo sapiens
tacattttgggcccacaaag

SEQ ID NO: 989 - DNA, 20 bp, homo sapiens
acattttgggcccacaaagt

SEQ ID NO: 990 - DNA, 20 bp, homo sapiens
gggcccacaaagtgggccgt

SEQ ID NO: 991 - DNA, 20 bp, homo sapiens
ggcccacaaagtgggccgtc

SEQ ID NO: 992 - DNA, 20 bp, homo sapiens
gcccacaaagtgggccgtcg

SEQ ID NO: 993 - DNA, 20 bp, homo sapiens
tccccgacggcccactttgt

SEQ ID NO: 994 - DNA, 20 bp, homo sapiens
atccccgacggcccactttg

SEQ ID NO: 995 - DNA, 20 bp, homo sapiens
ctctgtgcgctgatccccga

SEQ ID NO: 996 - DNA, 20 bp, homo sapiens
ggatcagcgcacagagttct

SEQ ID NO: 997 - DNA, 20 bp, homo sapiens
gatcagcgcacagagttctt

SEQ ID NO: 998 - DNA, 20 bp, homo sapiens
gttcttgggagcagcgccgt

SEQ ID NO: 999 - DNA, 20 bp, homo sapiens
ttcttgggagcagcgccgtt

SEQ ID NO: 1000 - DNA, 20 bp, homo sapiens
tcttgggagcagcgccgttg

SEQ ID NO: 1001 - DNA, 20 bp, homo sapiens
ggagagacagggggccccaa

SEQ ID NO: 1002 - DNA, 20 bp, homo sapiens
acatggggtggagagacagg

SEQ ID NO: 1003 - DNA, 20 bp, homo sapiens
gacatggggtggagagacag

SEQ ID NO: 1004 - DNA, 20 bp, homo sapiens
agacatggggtggagagaca

SEQ ID NO: 1005 - DNA, 20 bp, homo sapiens
gagacatggggtggagagac

SEQ ID NO: 1006 - DNA, 20 bp, homo sapiens
ttgaaggtggagacatgggg

SEQ ID NO: 1007 - DNA, 20 bp, homo sapiens
gtcttgaaggtggagacatg

SEQ ID NO: 1008 - DNA, 20 bp, homo sapiens
tgtcttgaaggtggagacat

SEQ ID NO: 1009 - DNA, 20 bp, homo sapiens
ttgtcttgaaggtggagaca

SEQ ID NO: 1010 - DNA, 20 bp, homo sapiens
atgtctccaccttcaagaca

SEQ ID NO: 1011 - DNA, 20 bp, homo sapiens
tgccacttaccttgtcttga

SEQ ID NO: 1012 - DNA, 20 bp, homo sapiens
cgggcttggcaggtctgcaa

SEQ ID NO: 1013 - DNA, 20 bp, homo sapiens
gggcttggcaggtctgcaaa

SEQ ID NO: 1014 - DNA, 20 bp, homo sapiens
ggcaggtctgcaaagggttt

SEQ ID NO: 1015 - DNA, 20 bp, homo sapiens
gcaggtctgcaaagggtttt

SEQ ID NO: 1016 - DNA, 20 bp, homo sapiens
caggtctgcaaagggttttg

SEQ ID NO: 1017 - DNA, 20 bp, homo sapiens
gcaaagggttttggggctcg

SEQ ID NO: 1018 - DNA, 20 bp, homo sapiens
aggcccagacgtgctgagtc

SEQ ID NO: 1019 - DNA, 20 bp, homo sapiens
tggccggactcagcacgtct

SEQ ID NO: 1020 - DNA, 20 bp, homo sapiens
atggccggactcagcacgtc

SEQ ID NO: 1021 - DNA, 20 bp, homo sapiens
agacgtgctgagtccggcca

SEQ ID NO: 1022 - DNA, 20 bp, homo sapiens
ttggagagggctaccatggc

SEQ ID NO: 1023 - DNA, 20 bp, homo sapiens
cttgttggagagggctacca

SEQ ID NO: 1024 - DNA, 20 bp, homo sapiens
cagcttcagcttgttggaga

SEQ ID NO: 1025 - DNA, 20 bp, homo sapiens
tcagcttcagcttgttggag

SEQ ID NO: 1026 - DNA, 20 bp, homo sapiens
tcgcttcagcttcagcttgt

SEQ ID NO: 1027 - DNA, 20 bp, homo sapiens
gctgaagctgaagcgacagc

SEQ ID NO: 1028 - DNA, 20 bp, homo sapiens
gtatgaagagcaagccttcc

SEQ ID NO: 1029 - DNA, 20 bp, homo sapiens
caagccttccaggacctgag

SEQ ID NO: 1030 - DNA, 20 bp, homo sapiens
aagccttccaggacctgagc

SEQ ID NO: 1031 - DNA, 20 bp, homo sapiens
agccttccaggacctgagcg

SEQ ID NO: 1032 - DNA, 20 bp, homo sapiens
caccccgctcaggtcctgga

SEQ ID NO: 1033 - DNA, 20 bp, homo sapiens
gactcaccccgctcaggtcc

SEQ ID NO: 1034 - DNA, 20 bp, homo sapiens
ggggatgactcaccccgctc

SEQ ID NO: 1035 - DNA, 20 bp, homo sapiens
tactcccagggggacccacc

SEQ ID NO: 1036 - DNA, 20 bp, homo sapiens
tcccagggggacccacctgg

SEQ ID NO: 1037 - DNA, 20 bp, homo sapiens
gccaccaggtgggtccccct

SEQ ID NO: 1038 - DNA, 20 bp, homo sapiens
tgccaccaggtgggtccccc

SEQ ID NO: 1039 - DNA, 20 bp, homo sapiens
gtgaggtgctgccaccaggt

SEQ ID NO: 1040 - DNA, 20 bp, homo sapiens
tgtgaggtgctgccaccagg

SEQ ID NO: 1041 - DNA, 20 bp, homo sapiens
aaatgtgaggtgctgccacc

SEQ ID NO: 1042 - DNA, 20 bp, homo sapiens
gcagcacctcacatttgatg

SEQ ID NO: 1043 - DNA, 20 bp, homo sapiens
cctcacatttgatgtggaaa

SEQ ID NO: 1044 - DNA, 20 bp, homo sapiens
ccgtttccacatcaaatgtg

SEQ ID NO: 1045 - DNA, 20 bp, homo sapiens
ggaaacggatgaagaacctc

SEQ ID NO: 1046 - DNA, 20 bp, homo sapiens
gaaacggatgaagaacctca

SEQ ID NO: 1047 - DNA, 20 bp, homo sapiens
aaacggatgaagaacctcag

SEQ ID NO: 1048 - DNA, 20 bp, homo sapiens
cggatgaagaacctcagggg

SEQ ID NO: 1049 - DNA, 20 bp, homo sapiens
ggatgaagaacctcaggggt

SEQ ID NO: 1050 - DNA, 20 bp, homo sapiens
aagggcagctcccacccctg

SEQ ID NO: 1051 - DNA, 20 bp, homo sapiens
tgggagctgccctttgatgc

SEQ ID NO: 1052 - DNA, 20 bp, homo sapiens
gtggcttgtccggcatcaaa

SEQ ID NO: 1053 - DNA, 20 bp, homo sapiens
agtggcttgtccggcatcaa

SEQ ID NO: 1054 - DNA, 20 bp, homo sapiens
tttgcgctcagtggcttgtc

SEQ ID NO: 1055 - DNA, 20 bp, homo sapiens
ttgggtacatttgcgctcag

SEQ ID NO: 1056 - DNA, 20 bp, homo sapiens
ctgagcgcaaatgtacccaa

SEQ ID NO: 1057 - DNA, 20 bp, homo sapiens
tgtggccgctgctcaccatt

SEQ ID NO: 1058 - DNA, 20 bp, homo sapiens
ctgtggccgctgctcaccat

SEQ ID NO: 1059 - DNA, 20 bp, homo sapiens
agttcacccaaaaccccatg

SEQ ID NO: 1060 - DNA, 20 bp, homo sapiens
gttcacccaaaaccccatga

SEQ ID NO: 1061 - DNA, 20 bp, homo sapiens
ttcacccaaaaccccatgag

SEQ ID NO: 1062 - DNA, 20 bp, homo sapiens
caggcccctcatggggtttt

SEQ ID NO: 1063 - DNA, 20 bp, homo sapiens
ccaaaaccccatgaggggcc

SEQ ID NO: 1064 - DNA, 20 bp, homo sapiens
ccaggcccctcatggggttt

SEQ ID NO: 1065 - DNA, 20 bp, homo sapiens
caaaaccccatgaggggcct

SEQ ID NO: 1066 - DNA, 20 bp, homo sapiens
gatggcccaggcccctcatg

SEQ ID NO: 1067 - DNA, 20 bp, homo sapiens
ggatggcccaggcccctcat

SEQ ID NO: 1068 - DNA, 20 bp, homo sapiens
gggatggcccaggcccctca

SEQ ID NO: 1069 - DNA, 20 bp, homo sapiens
gatgtctcaggggatggccc

SEQ ID NO: 1070 - DNA, 20 bp, homo sapiens
gcggcagatgtctcagggga

SEQ ID NO: 1071 - DNA, 20 bp, homo sapiens
ggcagcggcagatgtctcag

SEQ ID NO: 1072 - DNA, 20 bp, homo sapiens
tggcagcggcagatgtctca

SEQ ID NO: 1073 - DNA, 20 bp, homo sapiens
gtggcagcggcagatgtctc

SEQ ID NO: 1074 - DNA, 20 bp, homo sapiens
gcagatggaggctgtggcag

SEQ ID NO: 1075 - DNA, 20 bp, homo sapiens
ctgatggcagatggaggctg

SEQ ID NO: 1076 - DNA, 20 bp, homo sapiens
cctccatctgccatcagtcc

SEQ ID NO: 1077 - DNA, 20 bp, homo sapiens
ccgggactgatggcagatgg

SEQ ID NO: 1078 - DNA, 20 bp, homo sapiens
ctccatctgccatcagtccc

SEQ ID NO: 1079 - DNA, 20 bp, homo sapiens
tccatctgccatcagtcccg

SEQ ID NO: 1080 - DNA, 20 bp, homo sapiens
tccccgggactgatggcaga

SEQ ID NO: 1081 - DNA, 20 bp, homo sapiens
gctgttctccccgggactga

SEQ ID NO: 1082 - DNA, 20 bp, homo sapiens
ctgctcttgctgttctcccc

SEQ ID NO: 1083 - DNA, 20 bp, homo sapiens
ccggggagaacagcaagagc

SEQ ID NO: 1084 - DNA, 20 bp, homo sapiens
cctgctcttgctgttctccc

SEQ ID NO: 1085 - DNA, 20 bp, homo sapiens
gggtggcgtagcactgtggg

SEQ ID NO: 1086 - DNA, 20 bp, homo sapiens
tgggtggcgtagcactgtgg

SEQ ID NO: 1087 - DNA, 20 bp, homo sapiens
ctgggtggcgtagcactgtg

SEQ ID NO: 1088 - DNA, 20 bp, homo sapiens
actgggtggcgtagcactgt

SEQ ID NO: 1089 - DNA, 20 bp, homo sapiens
tactgggtggcgtagcactg

SEQ ID NO: 1090 - DNA, 20 bp, homo sapiens
gtgctacgccacccagtacc

SEQ ID NO: 1091 - DNA, 20 bp, homo sapiens
gctgtagtcctggtactggg

SEQ ID NO: 1092 - DNA, 20 bp, homo sapiens
caggctgtagtcctggtact

SEQ ID NO: 1093 - DNA, 20 bp, homo sapiens
acaggctgtagtcctggtac

SEQ ID NO: 1094 - DNA, 20 bp, homo sapiens
ctgacgacaggctgtagtcc

SEQ ID NO: 1095 - DNA, 20 bp, homo sapiens
cagcctgtcgtcagcccaca

SEQ ID NO: 1096 - DNA, 20 bp, homo sapiens
acaccttgtgggctgacgac

SEQ ID NO: 1097 - DNA, 20 bp, homo sapiens
tcgtcagcccacaaggtgtc

SEQ ID NO: 1098 - DNA, 20 bp, homo sapiens
tcagcccacaaggtgtcagg

SEQ ID NO: 1099 - DNA, 20 bp, homo sapiens
cagcccacaaggtgtcaggt

SEQ ID NO: 1100 - DNA, 20 bp, homo sapiens
acacccacctgacaccttgt

SEQ ID NO: 1101 - DNA, 20 bp, homo sapiens
cacacccacctgacaccttg

SEQ ID NO: 1102 - DNA, 20 bp, homo sapiens
accaacccttctttcaggca

SEQ ID NO: 1103 - DNA, 20 bp, homo sapiens
ttctttcaggcatggcaagc

SEQ ID NO: 1104 - DNA, 20 bp, homo sapiens
ggcatggcaagccggctgct

SEQ ID NO: 1105 - DNA, 20 bp, homo sapiens
gcatggcaagccggctgctc

SEQ ID NO: 1106 - DNA, 20 bp, homo sapiens
caaatgagggcccgagcagc

SEQ ID NO: 1107 - DNA, 20 bp, homo sapiens
agcaggtaggactcaaatga

SEQ ID NO: 1108 - DNA, 20 bp, homo sapiens
cagcaggtaggactcaaatg

SEQ ID NO: 1109 - DNA, 20 bp, homo sapiens
ggtcagttcgggcagcaggt

SEQ ID NO: 1110 - DNA, 20 bp, homo sapiens
atctggtcagttcgggcagc

SEQ ID NO: 1111 - DNA, 20 bp, homo sapiens
cagtcatatctggtcagttc

SEQ ID NO: 1112 - DNA, 20 bp, homo sapiens
acagtcatatctggtcagtt

SEQ ID NO: 1113 - DNA, 20 bp, homo sapiens
actgaccagatatgactgtg

SEQ ID NO: 1114 - DNA, 20 bp, homo sapiens
gttcacctcacagtcatatc

SEQ ID NO: 1115 - DNA, 20 bp, homo sapiens
tgaggtgaacgtgcccgtgc

SEQ ID NO: 1116 - DNA, 20 bp, homo sapiens
gaggtgaacgtgcccgtgct

SEQ ID NO: 1117 - DNA, 20 bp, homo sapiens
agcgtggagcttcccagcac

SEQ ID NO: 1118 - DNA, 20 bp, homo sapiens
gagcgtggagcttcccagca

SEQ ID NO: 1119 - DNA, 20 bp, homo sapiens
ggaagctccacgctcctgca

SEQ ID NO: 1120 - DNA, 20 bp, homo sapiens
agctccacgctcctgcaagg

SEQ ID NO: 1121 - DNA, 20 bp, homo sapiens
gctccacgctcctgcaagga

SEQ ID NO: 1122 - DNA, 20 bp, homo sapiens
ctccacgctcctgcaaggag

SEQ ID NO: 1123 - DNA, 20 bp, homo sapiens
gtcccctccttgcaggagcg

SEQ ID NO: 1124 - DNA, 20 bp, homo sapiens
tgaggaggtcccctccttgc

SEQ ID NO: 1125 - DNA, 20 bp, homo sapiens
aggggacctcctcagagccc

SEQ ID NO: 1126 - DNA, 20 bp, homo sapiens
cctcctcagagccctggacc

SEQ ID NO: 1127 - DNA, 20 bp, homo sapiens
cctggtccagggctctgagg

SEQ ID NO: 1128 - DNA, 20 bp, homo sapiens
tggcctggtccagggctctg

SEQ ID NO: 1129 - DNA, 20 bp, homo sapiens
ggctcaggtggcctggtcca

SEQ ID NO: 1130 - DNA, 20 bp, homo sapiens
tggctcaggtggcctggtcc

SEQ ID NO: 1131 - DNA, 20 bp, homo sapiens
tggaccaggccacctgagcc

SEQ ID NO: 1132 - DNA, 20 bp, homo sapiens
aaggcctggctcaggtggcc

SEQ ID NO: 1133 - DNA, 20 bp, homo sapiens
ggtagaaggcctggctcagg

SEQ ID NO: 1134 - DNA, 20 bp, homo sapiens
tctgagctgtgatcttgtct

SEQ ID NO: 1135 - DNA, 20 bp, homo sapiens
ccgcagcctataacaacttt

SEQ ID NO: 1136 - DNA, 20 bp, homo sapiens
ccgaaagttgttataggctg

SEQ ID NO: 1137 - DNA, 20 bp, homo sapiens
gctcttccgaaagttgttat

SEQ ID NO: 1138 - DNA, 20 bp, homo sapiens
taacaactttcggaagagca

SEQ ID NO: 1139 - DNA, 20 bp, homo sapiens
cggaagagcatggacagcat

SEQ ID NO: 1140 - DNA, 20 bp, homo sapiens
cataggaaagaagcaatatc

SEQ ID NO: 1141 - DNA, 20 bp, homo sapiens
aagcaatatcaggtccagca

SEQ ID NO: 1142 - DNA, 20 bp, homo sapiens
agcaatatcaggtccagcat

SEQ ID NO: 1143 - DNA, 20 bp, homo sapiens
tgtagctgcaggacccatgc

SEQ ID NO: 1144 - DNA, 20 bp, homo sapiens
caggaggaaagtgtagctgc

SEQ ID NO: 1145 - DNA, 20 bp, homo sapiens
cactttcctcctgccagaga

SEQ ID NO: 1146 - DNA, 20 bp, homo sapiens
agttgtccatctctggcagg

SEQ ID NO: 1147 - DNA, 20 bp, homo sapiens
ggcagttgtccatctctggc

SEQ ID NO: 1148 - DNA, 20 bp, homo sapiens
gagcggcagttgtccatctc

SEQ ID NO: 1149 - DNA, 20 bp, homo sapiens
cgtaggggctggaggaagag

SEQ ID NO: 1150 - DNA, 20 bp, homo sapiens
attggacacgtaggggctgg

SEQ ID NO: 1151 - DNA, 20 bp, homo sapiens
agcattggacacgtaggggc

SEQ ID NO: 1152 - DNA, 20 bp, homo sapiens
gcacagcattggacacgtag

SEQ ID NO: 1153 - DNA, 20 bp, homo sapiens
tgcacagcattggacacgta

SEQ ID NO: 1154 - DNA, 20 bp, homo sapiens
ctgcacagcattggacacgt

SEQ ID NO: 1155 - DNA, 20 bp, homo sapiens
acgtgtccaatgctgtgcag

SEQ ID NO: 1156 - DNA, 20 bp, homo sapiens
cgtgtccaatgctgtgcaga

SEQ ID NO: 1157 - DNA, 20 bp, homo sapiens
cgcgtccctctgcacagcat

SEQ ID NO: 1158 - DNA, 20 bp, homo sapiens
gccgctcgaatacgatgact

SEQ ID NO: 1159 - DNA, 20 bp, homo sapiens
accgagtcatcgtattcgag

SEQ ID NO: 1160 - DNA, 20 bp, homo sapiens
aatacgatgactcggtgcag

SEQ ID NO: 1161 - DNA, 20 bp, homo sapiens
ggtgcagaggctgcaagtgc

SEQ ID NO: 1162 - DNA, 20 bp, homo sapiens
gcaagtgctggagaacatca

SEQ ID NO: 1163 - DNA, 20 bp, homo sapiens
tcatggaaaacaacactcag

SEQ ID NO: 1164 - DNA, 20 bp, homo sapiens
caacactcagtggctaatga

SEQ ID NO: 1165 - DNA, 20 bp, homo sapiens
actcagtggctaatgaaggt

SEQ ID NO: 1166 - DNA, 20 bp, homo sapiens
ctagcttgagaattatatcc

SEQ ID NO: 1167 - DNA, 20 bp, homo sapiens
tttctttcttcatgttgtcc

SEQ ID NO: 1168 - DNA, 20 bp, homo sapiens
ggacaacatgaagaaagaaa

SEQ ID NO: 1169 - DNA, 20 bp, homo sapiens
gaatgcagtacagaaccaga

SEQ ID NO: 1170 - DNA, 20 bp, homo sapiens
tttctatcatcacagccgtc

SEQ ID NO: 1171 - DNA, 20 bp, homo sapiens
acggctgtgatgatagaaat

SEQ ID NO: 1172 - DNA, 20 bp, homo sapiens
cggctgtgatgatagaaata

SEQ ID NO: 1173 - DNA, 20 bp, homo sapiens
aaacctgttgaaccaaacag

SEQ ID NO: 1174 - DNA, 20 bp, homo sapiens
gctccgctgtttggttcaac

SEQ ID NO: 1175 - DNA, 20 bp, homo sapiens
accaaacagcggagcaaacg

SEQ ID NO: 1176 - DNA, 20 bp, homo sapiens
tccgcgtttgctccgctgtt

SEQ ID NO: 1177 - DNA, 20 bp, homo sapiens
aacgcggaagttaactgatg

SEQ ID NO: 1178 - DNA, 20 bp, homo sapiens
ctagcttgagaattatatcc

SEQ ID NO: 1179 - DNA, 20 bp, homo sapiens
tttctttcttcatgttgtcc

SEQ ID NO: 1180 - DNA, 20 bp, homo sapiens
ggacaacatgaagaaagaaa

SEQ ID NO: 1181 - DNA, 20 bp, homo sapiens
gaatgcagtacagaaccaga

SEQ ID NO: 1182 - DNA, 20 bp, homo sapiens
tttctatcatcacagccgtc

SEQ ID NO: 1183 - DNA, 20 bp, homo sapiens
acggctgtgatgatagaaat

SEQ ID NO: 1184 - DNA, 20 bp, homo sapiens
cggctgtgatgatagaaata

SEQ ID NO: 1185 - DNA, 20 bp, homo sapiens
aaacctgttgaaccaaacag

SEQ ID NO: 1186 - DNA, 20 bp, homo sapiens
gctccgctgtttggttcaac

SEQ ID NO: 1187 - DNA, 20 bp, homo sapiens
accaaacagcggagcaaacg

SEQ ID NO: 1188 - DNA, 20 bp, homo sapiens
tccgcgtttgctccgctgtt

SEQ ID NO: 1189 - DNA, 20 bp, homo sapiens
aacgcggaagttaactgatg

SEQ ID NO: 1190 - DNA, 20 bp, homo sapiens
tacaagtttcctagaaaaga

SEQ ID NO: 1191 - DNA, 20 bp, homo sapiens
tagctagcaccttcttttct

SEQ ID NO: 1192 - DNA, 20 bp, homo sapiens
agaaaagaaggtgctagcta

SEQ ID NO: 1193 - DNA, 20 bp, homo sapiens
cttcttttattgactgtagt

SEQ ID NO: 1194 - DNA, 20 bp, homo sapiens
agaagagaaagatcagctac

SEQ ID NO: 1195 - DNA, 20 bp, homo sapiens
ttcaatgatggaattttgct

SEQ ID NO: 1196 - DNA, 20 bp, homo sapiens
tttttctagttcttcaatga

SEQ ID NO: 1197 - DNA, 20 bp, homo sapiens
aaaaaaaatagtgactgcca

SEQ ID NO: 1198 - DNA, 20 bp, homo sapiens
aagaactgaattattcaccg

SEQ ID NO: 1199 - DNA, 20 bp, homo sapiens
gaagcagcaacatgatctca

SEQ ID NO: 1200 - DNA, 20 bp, homo sapiens
tgtaaacttacagtttgatg

SEQ ID NO: 1201 - DNA, 20 bp, homo sapiens
ctattttttaaaagcagcta

SEQ ID NO: 1202 - DNA, 20 bp, homo sapiens
gttcttctttagcaacagtg

SEQ ID NO: 1203 - DNA, 20 bp, homo sapiens
tgttcttctttagcaacagt

SEQ ID NO: 1204 - DNA, 20 bp, homo sapiens
ttgttcttctttagcaacag

SEQ ID NO: 1205 - DNA, 20 bp, homo sapiens
tgtgctgaagtattcaaatc

SEQ ID NO: 1206 - DNA, 20 bp, homo sapiens
aaatcaggacacaccacgaa

SEQ ID NO: 1207 - DNA, 20 bp, homo sapiens
taacgtgtagatgccattcg

SEQ ID NO: 1208 - DNA, 20 bp, homo sapiens
tgatctcttctgtagaatta

SEQ ID NO: 1209 - DNA, 20 bp, homo sapiens
ttgatctcttctgtagaatt

SEQ ID NO: 1210 - DNA, 20 bp, homo sapiens
taattctacagaagagatca

SEQ ID NO: 1211 - DNA, 20 bp, homo sapiens
ctacagaagagatcaaggtg

SEQ ID NO: 1212 - DNA, 20 bp, homo sapiens
tttgcaggcctactgtgaca

SEQ ID NO: 1213 - DNA, 20 bp, homo sapiens
gcctactgtgacatggaagc

SEQ ID NO: 1214 - DNA, 20 bp, homo sapiens
tccagcttccatgtcacagt

SEQ ID NO: 1215 - DNA, 20 bp, homo sapiens
tactgtgacatggaagctgg

SEQ ID NO: 1216 - DNA, 20 bp, homo sapiens
tgtgacatggaagctggagg

SEQ ID NO: 1217 - DNA, 20 bp, homo sapiens
gacatggaagctggaggagg

SEQ ID NO: 1218 - DNA, 20 bp, homo sapiens
acatggaagctggaggaggc

SEQ ID NO: 1219 - DNA, 20 bp, homo sapiens
tggaagctggaggaggcggg

SEQ ID NO: 1220 - DNA, 20 bp, homo sapiens
gacaattattcagcgacgtg

SEQ ID NO: 1221 - DNA, 20 bp, homo sapiens
attattcagcgacgtgagga

SEQ ID NO: 1222 - DNA, 20 bp, homo sapiens
atggcagcgttgattttcag

SEQ ID NO: 1223 - DNA, 20 bp, homo sapiens
gcgttgattttcagaggact

SEQ ID NO: 1224 - DNA, 20 bp, homo sapiens
gacttggaaagaatataaag

SEQ ID NO: 1225 - DNA, 20 bp, homo sapiens
ggaaagaatataaagtggta

SEQ ID NO: 1226 - DNA, 20 bp, homo sapiens
cagggatttggtaacccttc

SEQ ID NO: 1227 - DNA, 20 bp, homo sapiens
gtaacccttcaggagaatat

SEQ ID NO: 1228 - DNA, 20 bp, homo sapiens
cccttcaggagaatattggc

SEQ ID NO: 1229 - DNA, 20 bp, homo sapiens
ccagccaatattctcctgaa

SEQ ID NO: 1230 - DNA, 20 bp, homo sapiens
ccttcaggagaatattggct

SEQ ID NO: 1231 - DNA, 20 bp, homo sapiens
cccagccaatattctcctga

SEQ ID NO: 1232 - DNA, 20 bp, homo sapiens
ttaaaatacaccttaaagac

SEQ ID NO: 1233 - DNA, 20 bp, homo sapiens
taaaatacaccttaaagact

SEQ ID NO: 1234 - DNA, 20 bp, homo sapiens
atacaccttaaagactggga

SEQ ID NO: 1235 - DNA, 20 bp, homo sapiens
tacaccttaaagactgggaa

SEQ ID NO: 1236 - DNA, 20 bp, homo sapiens
cattcccttcccagtcttta

SEQ ID NO: 1237 - DNA, 20 bp, homo sapiens
taaagactgggaagggaatg

SEQ ID NO: 1238 - DNA, 20 bp, homo sapiens
caagtgaagaactcaattat

SEQ ID NO: 1239 - DNA, 20 bp, homo sapiens
gcttacaggattcaccttaa

SEQ ID NO: 1240 - DNA, 20 bp, homo sapiens
attcaccttaaaggacttac

SEQ ID NO: 1241 - DNA, 20 bp, homo sapiens
ttcaccttaaaggacttaca

SEQ ID NO: 1242 - DNA, 20 bp, homo sapiens
ctgtccctgtaagtccttta

SEQ ID NO: 1243 - DNA, 20 bp, homo sapiens
aaaggacttacagggacagc

SEQ ID NO: 1244 - DNA, 20 bp, homo sapiens
gctgatgctgcttattttgc

SEQ ID NO: 1245 - DNA, 20 bp, homo sapiens
ataagcagcatcagccaacc

SEQ ID NO: 1246 - DNA, 20 bp, homo sapiens
tgctaaaatcatttcctggt

SEQ ID NO: 1247 - DNA, 20 bp, homo sapiens
tttgtgctaaaatcatttcc

SEQ ID NO: 1248 - DNA, 20 bp, homo sapiens
aggaaatgattttagcacaa

SEQ ID NO: 1249 - DNA, 20 bp, homo sapiens
aatgattttagcacaaagga

SEQ ID NO: 1250 - DNA, 20 bp, homo sapiens
aaatgttcacaaatgctaac

SEQ ID NO: 1251 - DNA, 20 bp, homo sapiens
tgttcacaaatgctaacagg

SEQ ID NO: 1252 - DNA, 20 bp, homo sapiens
cacaaatgctaacaggaggt

SEQ ID NO: 1253 - DNA, 20 bp, homo sapiens
acaaatgctaacaggaggta

SEQ ID NO: 1254 - DNA, 20 bp, homo sapiens
ggctggtggtttgatgcatg

SEQ ID NO: 1255 - DNA, 20 bp, homo sapiens
tgtggtccttccaacttgaa

SEQ ID NO: 1256 - DNA, 20 bp, homo sapiens
tacattccgttcaagttgga

SEQ ID NO: 1257 - DNA, 20 bp, homo sapiens
atagtacattccgttcaagt

SEQ ID NO: 1258 - DNA, 20 bp, homo sapiens
acggaatgtactatccacag

SEQ ID NO: 1259 - DNA, 20 bp, homo sapiens
ttatttgtgttctgcctctg

SEQ ID NO: 1260 - DNA, 20 bp, homo sapiens
cagaacacaaataagttcaa

SEQ ID NO: 1261 - DNA, 20 bp, homo sapiens
ataagttcaacggcattaaa

SEQ ID NO: 1262 - DNA, 20 bp, homo sapiens
acggcattaaatggtactac

SEQ ID NO: 1263 - DNA, 20 bp, homo sapiens
attaaatggtactactggaa

SEQ ID NO: 1264 - DNA, 20 bp, homo sapiens
tggtactactggaaaggctc

SEQ ID NO: 1265 - DNA, 20 bp, homo sapiens
aggctcaggctattcgctca

SEQ ID NO: 1266 - DNA, 20 bp, homo sapiens
tggtcggatcatcatggttg

SEQ ID NO: 1267 - DNA, 20 bp, homo sapiens
atctgctggtcggatcatca

SEQ ID NO: 1268 - DNA, 20 bp, homo sapiens
atgtttagaaatctgctggt

SEQ ID NO: 1269 - DNA, 20 bp, homo sapiens
tgggatgtttagaaatctgc

SEQ ID NO: 1270 - DNA, 20 bp, homo sapiens
aggctacctaagaggatgag

SEQ ID NO: 1271 - DNA, 20 bp, homo sapiens
gaggatgagcggtgctccga

SEQ ID NO: 1272 - DNA, 20 bp, homo sapiens
atgagcggtgctccgacggc

SEQ ID NO: 1273 - DNA, 20 bp, homo sapiens
tgagcggtgctccgacggcc

SEQ ID NO: 1274 - DNA, 20 bp, homo sapiens
gagcggtgctccgacggccg

SEQ ID NO: 1275 - DNA, 20 bp, homo sapiens
atcagggctgccccggccgt

SEQ ID NO: 1276 - DNA, 20 bp, homo sapiens
gcagagcatcagggctgccc

SEQ ID NO: 1277 - DNA, 20 bp, homo sapiens
ggtggcggcgcagagcatca

SEQ ID NO: 1278 - DNA, 20 bp, homo sapiens
cggtggcggcgcagagcatc

SEQ ID NO: 1279 - DNA, 20 bp, homo sapiens
gctcagtagcacggcggtgg

SEQ ID NO: 1280 - DNA, 20 bp, homo sapiens
agcgctcagtagcacggcgg

SEQ ID NO: 1281 - DNA, 20 bp, homo sapiens
ctgagcgctcagtagcacgg

SEQ ID NO: 1282 - DNA, 20 bp, homo sapiens
cgccgtgctactgagcgctc

SEQ ID NO: 1283 - DNA, 20 bp, homo sapiens
gccgtgctactgagcgctca

SEQ ID NO: 1284 - DNA, 20 bp, homo sapiens
gccctgagcgctcagtagca

SEQ ID NO: 1285 - DNA, 20 bp, homo sapiens
gtgctactgagcgctcaggg

SEQ ID NO: 1286 - DNA, 20 bp, homo sapiens
cgcggcgacttggactgcac

SEQ ID NO: 1287 - DNA, 20 bp, homo sapiens
gcgcggcgacttggactgca

SEQ ID NO: 1288 - DNA, 20 bp, homo sapiens
ggacgcaaagcgcggcgact

SEQ ID NO: 1289 - DNA, 20 bp, homo sapiens
agtcgccgcgctttgcgtcc

SEQ ID NO: 1290 - DNA, 20 bp, homo sapiens
gtcgccgcgctttgcgtcct

SEQ ID NO: 1291 - DNA, 20 bp, homo sapiens
tcgtcccaggacgcaaagcg

SEQ ID NO: 1292 - DNA, 20 bp, homo sapiens
caggacattcatctcgtccc

SEQ ID NO: 1293 - DNA, 20 bp, homo sapiens
ctgggacgagatgaatgtcc

SEQ ID NO: 1294 - DNA, 20 bp, homo sapiens
gagatgaatgtcctggcgca

SEQ ID NO: 1295 - DNA, 20 bp, homo sapiens
gctgcaggagtccgtgcgcc

SEQ ID NO: 1296 - DNA, 20 bp, homo sapiens
gcgcacggactcctgcagct

SEQ ID NO: 1297 - DNA, 20 bp, homo sapiens
cggactcctgcagctcggcc

SEQ ID NO: 1298 - DNA, 20 bp, homo sapiens
ggactcctgcagctcggcca

SEQ ID NO: 1299 - DNA, 20 bp, homo sapiens
gactcctgcagctcggccag

SEQ ID NO: 1300 - DNA, 20 bp, homo sapiens
gcagcccctggccgagctgc

SEQ ID NO: 1301 - DNA, 20 bp, homo sapiens
ccaggggctgcgcgaacacg

SEQ ID NO: 1302 - DNA, 20 bp, homo sapiens
ccgcgtgttcgcgcagcccc

SEQ ID NO: 1303 - DNA, 20 bp, homo sapiens
cagcgcgctcagctgactgc

SEQ ID NO: 1304 - DNA, 20 bp, homo sapiens
ccgcagtcagctgagcgcgc

SEQ ID NO: 1305 - DNA, 20 bp, homo sapiens
ccagcgcgctcagctgactg

SEQ ID NO: 1306 - DNA, 20 bp, homo sapiens
gtcagctgagcgcgctggag

SEQ ID NO: 1307 - DNA, 20 bp, homo sapiens
gagcggcgcctgagcgcgtg

SEQ ID NO: 1308 - DNA, 20 bp, homo sapiens
agcggcgcctgagcgcgtgc

SEQ ID NO: 1309 - DNA, 20 bp, homo sapiens
aggcggacccgcacgcgctc

SEQ ID NO: 1310 - DNA, 20 bp, homo sapiens
cgcgtgcgggtccgcctgtc

SEQ ID NO: 1311 - DNA, 20 bp, homo sapiens
gcgtgcgggtccgcctgtca

SEQ ID NO: 1312 - DNA, 20 bp, homo sapiens
gtccgcctgtcagggaaccg

SEQ ID NO: 1313 - DNA, 20 bp, homo sapiens
tccgcctgtcagggaaccga

SEQ ID NO: 1314 - DNA, 20 bp, homo sapiens
ccgcctgtcagggaaccgag

SEQ ID NO: 1315 - DNA, 20 bp, homo sapiens
cccctcggttccctgacagg

SEQ ID NO: 1316 - DNA, 20 bp, homo sapiens
ggacccctcggttccctgac

SEQ ID NO: 1317 - DNA, 20 bp, homo sapiens
cgggaggtcggtggacccct

SEQ ID NO: 1318 - DNA, 20 bp, homo sapiens
aggggctaacgggaggtcgg

SEQ ID NO: 1319 - DNA, 20 bp, homo sapiens
ctcaggggctaacgggaggt

SEQ ID NO: 1320 - DNA, 20 bp, homo sapiens
ggctctcaggggctaacggg

SEQ ID NO: 1321 - DNA, 20 bp, homo sapiens
tcccgttagcccctgagagc

SEQ ID NO: 1322 - DNA, 20 bp, homo sapiens
cccgttagcccctgagagcc

SEQ ID NO: 1323 - DNA, 20 bp, homo sapiens
cccggctctcaggggctaac

SEQ ID NO: 1324 - DNA, 20 bp, homo sapiens
acccggctctcaggggctaa

SEQ ID NO: 1325 - DNA, 20 bp, homo sapiens
gttagcccctgagagccggg

SEQ ID NO: 1326 - DNA, 20 bp, homo sapiens
agggtccacccggctctcag

SEQ ID NO: 1327 - DNA, 20 bp, homo sapiens
cagggtccacccggctctca

SEQ ID NO: 1328 - DNA, 20 bp, homo sapiens
tcagggtccacccggctctc

SEQ ID NO: 1329 - DNA, 20 bp, homo sapiens
tgagagccgggtggaccctg

SEQ ID NO: 1330 - DNA, 20 bp, homo sapiens
gaaggacctcagggtccacc

SEQ ID NO: 1331 - DNA, 20 bp, homo sapiens
gcaggctgtgaaggacctca

SEQ ID NO: 1332 - DNA, 20 bp, homo sapiens
tgcaggctgtgaaggacctc

SEQ ID NO: 1333 - DNA, 20 bp, homo sapiens
tgaggtccttcacagcctgc

SEQ ID NO: 1334 - DNA, 20 bp, homo sapiens
cacgtacctgcaggctgtga

SEQ ID NO: 1335 - DNA, 20 bp, homo sapiens
ccctggggacacgtacctgc

SEQ ID NO: 1336 - DNA, 20 bp, homo sapiens
ccctccccagacacaactca

SEQ ID NO: 1337 - DNA, 20 bp, homo sapiens
tgagccttgagttgtgtctg

SEQ ID NO: 1338 - DNA, 20 bp, homo sapiens
ctgagccttgagttgtgtct

SEQ ID NO: 1339 - DNA, 20 bp, homo sapiens
tctgagccttgagttgtgtc

SEQ ID NO: 1340 - DNA, 20 bp, homo sapiens
aactcaaggctcagaacagc

SEQ ID NO: 1341 - DNA, 20 bp, homo sapiens
gatccagcaactcttccaca

SEQ ID NO: 1342 - DNA, 20 bp, homo sapiens
ccagcaactcttccacaagg

SEQ ID NO: 1343 - DNA, 20 bp, homo sapiens
ccaccttgtggaagagttgc

SEQ ID NO: 1344 - DNA, 20 bp, homo sapiens
gctgctgctgggccaccttg

SEQ ID NO: 1345 - DNA, 20 bp, homo sapiens
acaaggtggcccagcagcag

SEQ ID NO: 1346 - DNA, 20 bp, homo sapiens
ggcccagcagcagcggcacc

SEQ ID NO: 1347 - DNA, 20 bp, homo sapiens
ctccaggtgccgctgctgct

SEQ ID NO: 1348 - DNA, 20 bp, homo sapiens
tctccaggtgccgctgctgc

SEQ ID NO: 1349 - DNA, 20 bp, homo sapiens
ttcgcaggtgctgcttctcc

SEQ ID NO: 1350 - DNA, 20 bp, homo sapiens
tttgcagatgctgaattcgc

SEQ ID NO: 1351 - DNA, 20 bp, homo sapiens
aattcagcatctgcaaagcc

SEQ ID NO: 1352 - DNA, 20 bp, homo sapiens
cccttgatcctagggttacc

SEQ ID NO: 1353 - DNA, 20 bp, homo sapiens
cccatcctagtttggcctcc

SEQ ID NO: 1354 - DNA, 20 bp, homo sapiens
gtggtccaggaggccaaact

SEQ ID NO: 1355 - DNA, 20 bp, homo sapiens
ctaggtgcttgtggtccagg

SEQ ID NO: 1356 - DNA, 20 bp, homo sapiens
ggtctaggtgcttgtggtcc

SEQ ID NO: 1357 - DNA, 20 bp, homo sapiens
ccacaagcacctagaccatg

SEQ ID NO: 1358 - DNA, 20 bp, homo sapiens
cctcatggtctaggtgcttg

SEQ ID NO: 1359 - DNA, 20 bp, homo sapiens
caagcacctagaccatgagg

SEQ ID NO: 1360 - DNA, 20 bp, homo sapiens
gcttggccacctcatggtct

SEQ ID NO: 1361 - DNA, 20 bp, homo sapiens
gggcaggcttggccacctca

SEQ ID NO: 1362 - DNA, 20 bp, homo sapiens
ccaagcctgcccgaagaaag

SEQ ID NO: 1363 - DNA, 20 bp, homo sapiens
cctctttcttcgggcaggct

SEQ ID NO: 1364 - DNA, 20 bp, homo sapiens
ggcagcctctttcttcgggc

SEQ ID NO: 1365 - DNA, 20 bp, homo sapiens
ctcgggcagcctctttcttc

SEQ ID NO: 1366 - DNA, 20 bp, homo sapiens
tctcgggcagcctctttctt

SEQ ID NO: 1367 - DNA, 20 bp, homo sapiens
aagaaagaggctgcccgaga

SEQ ID NO: 1368 - DNA, 20 bp, homo sapiens
tcaactggctgggccatctc

SEQ ID NO: 1369 - DNA, 20 bp, homo sapiens
gtcaactggctgggccatct

SEQ ID NO: 1370 - DNA, 20 bp, homo sapiens
gatggcccagccagttgacc

SEQ ID NO: 1371 - DNA, 20 bp, homo sapiens
gtgagccgggtcaactggct

SEQ ID NO: 1372 - DNA, 20 bp, homo sapiens
tgtgagccgggtcaactggc

SEQ ID NO: 1373 - DNA, 20 bp, homo sapiens
acattgtgagccgggtcaac

SEQ ID NO: 1374 - DNA, 20 bp, homo sapiens
ggcggctgacattgtgagcc

SEQ ID NO: 1375 - DNA, 20 bp, homo sapiens
aggcggctgacattgtgagc

SEQ ID NO: 1376 - DNA, 20 bp, homo sapiens
gcagacactcacggtgcagg

SEQ ID NO: 1377 - DNA, 20 bp, homo sapiens
ggggcagacactcacggtgc

SEQ ID NO: 1378 - DNA, 20 bp, homo sapiens
atctcccttcagggctgccc

SEQ ID NO: 1379 - DNA, 20 bp, homo sapiens
tctcccttcagggctgccca

SEQ ID NO: 1380 - DNA, 20 bp, homo sapiens
agggctgcccagggattgcc

SEQ ID NO: 1381 - DNA, 20 bp, homo sapiens
aacagctcctggcaatccct

SEQ ID NO: 1382 - DNA, 20 bp, homo sapiens
gaacagctcctggcaatccc

SEQ ID NO: 1383 - DNA, 20 bp, homo sapiens
ggattgccaggagctgttcc

SEQ ID NO: 1384 - DNA, 20 bp, homo sapiens
tgccaggagctgttccaggt

SEQ ID NO: 1385 - DNA, 20 bp, homo sapiens
ccaggagctgttccaggttg

SEQ ID NO: 1386 - DNA, 20 bp, homo sapiens
ccccaacctggaacagctcc

SEQ ID NO: 1387 - DNA, 20 bp, homo sapiens
agctgttccaggttggggag

SEQ ID NO: 1388 - DNA, 20 bp, homo sapiens
cactctgcctctccccaacc

SEQ ID NO: 1389 - DNA, 20 bp, homo sapiens
caggttggggagaggcagag

SEQ ID NO: 1390 - DNA, 20 bp, homo sapiens
actatttgaaatccagcctc

SEQ ID NO: 1391 - DNA, 20 bp, homo sapiens
ctatttgaaatccagcctca

SEQ ID NO: 1392 - DNA, 20 bp, homo sapiens
tatttgaaatccagcctcag

SEQ ID NO: 1393 - DNA, 20 bp, homo sapiens
atggcggagacccctgaggc

SEQ ID NO: 1394 - DNA, 20 bp, homo sapiens
aaaaatggcggagacccctg

SEQ ID NO: 1395 - DNA, 20 bp, homo sapiens
tcaggggtctccgccatttt

SEQ ID NO: 1396 - DNA, 20 bp, homo sapiens
ttgcagttcaccaaaaatgg

SEQ ID NO: 1397 - DNA, 20 bp, homo sapiens
atcttgcagttcaccaaaaa

SEQ ID NO: 1398 - DNA, 20 bp, homo sapiens
gtgaactgcaagatgacctc

SEQ ID NO: 1399 - DNA, 20 bp, homo sapiens
actgcaagatgacctcaggt

SEQ ID NO: 1400 - DNA, 20 bp, homo sapiens
ctgcaagatgacctcaggta

SEQ ID NO: 1401 - DNA, 20 bp, homo sapiens
ggactaacacaccctacctg

SEQ ID NO: 1402 - DNA, 20 bp, homo sapiens
gtacctttctgggcagatgg

SEQ ID NO: 1403 - DNA, 20 bp, homo sapiens
ctttctgggcagatggaggc

SEQ ID NO: 1404 - DNA, 20 bp, homo sapiens
gaggctggacagtaattcag

SEQ ID NO: 1405 - DNA, 20 bp, homo sapiens
gtaattcagaggcgccacga

SEQ ID NO: 1406 - DNA, 20 bp, homo sapiens
gaggcgccacgatggctcag

SEQ ID NO: 1407 - DNA, 20 bp, homo sapiens
tgaagtccactgagccatcg

SEQ ID NO: 1408 - DNA, 20 bp, homo sapiens
atggctcagtggacttcaac

SEQ ID NO: 1409 - DNA, 20 bp, homo sapiens
cagtggacttcaaccggccc

SEQ ID NO: 1410 - DNA, 20 bp, homo sapiens
agtggacttcaaccggccct

SEQ ID NO: 1411 - DNA, 20 bp, homo sapiens
ccggccctgggaagcctaca

SEQ ID NO: 1412 - DNA, 20 bp, homo sapiens
ccttgtaggcttcccagggc

SEQ ID NO: 1413 - DNA, 20 bp, homo sapiens
gccctgggaagcctacaagg

SEQ ID NO: 1414 - DNA, 20 bp, homo sapiens
ccctgggaagcctacaaggc

SEQ ID NO: 1415 - DNA, 20 bp, homo sapiens
cccgccttgtaggcttccca

SEQ ID NO: 1416 - DNA, 20 bp, homo sapiens
cctgggaagcctacaaggcg

SEQ ID NO: 1417 - DNA, 20 bp, homo sapiens
ccccgccttgtaggcttccc

SEQ ID NO: 1418 - DNA, 20 bp, homo sapiens
gaagcctacaaggcggggtt

SEQ ID NO: 1419 - DNA, 20 bp, homo sapiens
aagcctacaaggcggggttt

SEQ ID NO: 1420 - DNA, 20 bp, homo sapiens
agcctacaaggcggggtttg

SEQ ID NO: 1421 - DNA, 20 bp, homo sapiens
atccccaaaccccgccttgt

SEQ ID NO: 1422 - DNA, 20 bp, homo sapiens
gcggggtttggggatcccca

SEQ ID NO: 1423 - DNA, 20 bp, homo sapiens
ggtttggggatccccacggt

SEQ ID NO: 1424 - DNA, 20 bp, homo sapiens
cactagaaacacctaccgtg

SEQ ID NO: 1425 - DNA, 20 bp, homo sapiens
ccactagaaacacctaccgt

SEQ ID NO: 1426 - DNA, 20 bp, homo sapiens
ctcccactccaggcgagttc

SEQ ID NO: 1427 - DNA, 20 bp, homo sapiens
cactccaggcgagttctggc

SEQ ID NO: 1428 - DNA, 20 bp, homo sapiens
actccaggcgagttctggct

SEQ ID NO: 1429 - DNA, 20 bp, homo sapiens
agacccagccagaactcgcc

SEQ ID NO: 1430 - DNA, 20 bp, homo sapiens
aggcgagttctggctgggtc

SEQ ID NO: 1431 - DNA, 20 bp, homo sapiens
gttctggctgggtctggaga

SEQ ID NO: 1432 - DNA, 20 bp, homo sapiens
ggagaaggtgcatagcatca

SEQ ID NO: 1433 - DNA, 20 bp, homo sapiens
gagaaggtgcatagcatcac

SEQ ID NO: 1434 - DNA, 20 bp, homo sapiens
agaaggtgcatagcatcacg

SEQ ID NO: 1435 - DNA, 20 bp, homo sapiens
gaaggtgcatagcatcacgg

SEQ ID NO: 1436 - DNA, 20 bp, homo sapiens
gggggaccgcaacagccgcc

SEQ ID NO: 1437 - DNA, 20 bp, homo sapiens
gcacggccaggcggctgttg

SEQ ID NO: 1438 - DNA, 20 bp, homo sapiens
gccgcctggccgtgcagctg

SEQ ID NO: 1439 - DNA, 20 bp, homo sapiens
ccgcctggccgtgcagctgc

SEQ ID NO: 1440 - DNA, 20 bp, homo sapiens
cccgcagctgcacggccagg

SEQ ID NO: 1441 - DNA, 20 bp, homo sapiens
agtcccgcagctgcacggcc

SEQ ID NO: 1442 - DNA, 20 bp, homo sapiens
tggccgtgcagctgcgggac

SEQ ID NO: 1443 - DNA, 20 bp, homo sapiens
ggccgtgcagctgcgggact

SEQ ID NO: 1444 - DNA, 20 bp, homo sapiens
atcccagtcccgcagctgca

SEQ ID NO: 1445 - DNA, 20 bp, homo sapiens
gtgcagctgcgggactggga

SEQ ID NO: 1446 - DNA, 20 bp, homo sapiens
cacggagaactgcagcaact

SEQ ID NO: 1447 - DNA, 20 bp, homo sapiens
gctgcagttctccgtgcacc

SEQ ID NO: 1448 - DNA, 20 bp, homo sapiens
ctgcagttctccgtgcacct

SEQ ID NO: 1449 - DNA, 20 bp, homo sapiens
cagttctccgtgcacctggg

SEQ ID NO: 1450 - DNA, 20 bp, homo sapiens
ctccgtgcacctgggtggcg

SEQ ID NO: 1451 - DNA, 20 bp, homo sapiens
gtcctcgccacccaggtgca

SEQ ID NO: 1452 - DNA, 20 bp, homo sapiens
gcacctgggtggcgaggaca

SEQ ID NO: 1453 - DNA, 20 bp, homo sapiens
aggccgtgtcctcgccaccc

SEQ ID NO: 1454 - DNA, 20 bp, homo sapiens
tgcagtgagctgcaggctat

SEQ ID NO: 1455 - DNA, 20 bp, homo sapiens
cctgcagctcactgcacccg

SEQ ID NO: 1456 - DNA, 20 bp, homo sapiens
ccacgggtgcagtgagctgc

SEQ ID NO: 1457 - DNA, 20 bp, homo sapiens
cagctcactgcacccgtggc

SEQ ID NO: 1458 - DNA, 20 bp, homo sapiens
tgcacccgtggccggccagc

SEQ ID NO: 1459 - DNA, 20 bp, homo sapiens
gcacccgtggccggccagct

SEQ ID NO: 1460 - DNA, 20 bp, homo sapiens
gcgcccagctggccggccac

SEQ ID NO: 1461 - DNA, 20 bp, homo sapiens
ggcgcccagctggccggcca

SEQ ID NO: 1462 - DNA, 20 bp, homo sapiens
ggtggtggcgcccagctggc

SEQ ID NO: 1463 - DNA, 20 bp, homo sapiens
ggacggtggtggcgcccagc

SEQ ID NO: 1464 - DNA, 20 bp, homo sapiens
gccaccaccgtcccacccag

SEQ ID NO: 1465 - DNA, 20 bp, homo sapiens
gccgctgggtgggacggtgg

SEQ ID NO: 1466 - DNA, 20 bp, homo sapiens
gaggccgctgggtgggacgg

SEQ ID NO: 1467 - DNA, 20 bp, homo sapiens
ggagaggccgctgggtggga

SEQ ID NO: 1468 - DNA, 20 bp, homo sapiens
gtacggagaggccgctgggt

SEQ ID NO: 1469 - DNA, 20 bp, homo sapiens
ggtacggagaggccgctggg

SEQ ID NO: 1470 - DNA, 20 bp, homo sapiens
aagggtacggagaggccgct

SEQ ID NO: 1471 - DNA, 20 bp, homo sapiens
gaagggtacggagaggccgc

SEQ ID NO: 1472 - DNA, 20 bp, homo sapiens
aagtggagaagggtacggag

SEQ ID NO: 1473 - DNA, 20 bp, homo sapiens
tctccgtacccttctccact

SEQ ID NO: 1474 - DNA, 20 bp, homo sapiens
ctccgtacccttctccactt

SEQ ID NO: 1475 - DNA, 20 bp, homo sapiens
gtcccaagtggagaagggta

SEQ ID NO: 1476 - DNA, 20 bp, homo sapiens
acccttctccacttgggacc

SEQ ID NO: 1477 - DNA, 20 bp, homo sapiens
tcctggtcccaagtggagaa

SEQ ID NO: 1478 - DNA, 20 bp, homo sapiens
atcctggtcccaagtggaga

SEQ ID NO: 1479 - DNA, 20 bp, homo sapiens
gtcgtgatcctggtcccaag

SEQ ID NO: 1480 - DNA, 20 bp, homo sapiens
accaggatcacgacctccgc

SEQ ID NO: 1481 - DNA, 20 bp, homo sapiens
ccaggatcacgacctccgca

SEQ ID NO: 1482 - DNA, 20 bp, homo sapiens
ccctgcggaggtcgtgatcc

SEQ ID NO: 1483 - DNA, 20 bp, homo sapiens
cgcagttcttgtccctgcgg

SEQ ID NO: 1484 - DNA, 20 bp, homo sapiens
tggcgcagttcttgtccctg

SEQ ID NO: 1485 - DNA, 20 bp, homo sapiens
aactgcgccaagagcctctc

SEQ ID NO: 1486 - DNA, 20 bp, homo sapiens
ctgctcaccagagaggctct

SEQ ID NO: 1487 - DNA, 20 bp, homo sapiens
gcagggcctgctcaccagag

SEQ ID NO: 1488 - DNA, 20 bp, homo sapiens
ccctgaccccggcaggaggc

SEQ ID NO: 1489 - DNA, 20 bp, homo sapiens
tgaccccggcaggaggctgg

SEQ ID NO: 1490 - DNA, 20 bp, homo sapiens
ccggcaggaggctggtggtt

SEQ ID NO: 1491 - DNA, 20 bp, homo sapiens
gttgaggttggaatggctgc

SEQ ID NO: 1492 - DNA, 20 bp, homo sapiens
tgcagccattccaacctcaa

SEQ ID NO: 1493 - DNA, 20 bp, homo sapiens
actggccgttgaggttggaa

SEQ ID NO: 1494 - DNA, 20 bp, homo sapiens
gaagtactggccgttgaggt

SEQ ID NO: 1495 - DNA, 20 bp, homo sapiens
agcggaagtactggccgttg

SEQ ID NO: 1496 - DNA, 20 bp, homo sapiens
gtgggatggagcggaagtac

SEQ ID NO: 1497 - DNA, 20 bp, homo sapiens
tccgctccatcccacagcag

SEQ ID NO: 1498 - DNA, 20 bp, homo sapiens
gccgctgctgtgggatggag

SEQ ID NO: 1499 - DNA, 20 bp, homo sapiens
cttctgccgctgctgtggga

SEQ ID NO: 1500 - DNA, 20 bp, homo sapiens
taagcttctgccgctgctgt

SEQ ID NO: 1501 - DNA, 20 bp, homo sapiens
ttaagcttctgccgctgctg

SEQ ID NO: 1502 - DNA, 20 bp, homo sapiens
gcagcggcagaagcttaaga

SEQ ID NO: 1503 - DNA, 20 bp, homo sapiens
cagcggcagaagcttaagaa

SEQ ID NO: 1504 - DNA, 20 bp, homo sapiens
agcttaagaagggaatcttc

SEQ ID NO: 1505 - DNA, 20 bp, homo sapiens
agggaatcttctggaagacc

SEQ ID NO: 1506 - DNA, 20 bp, homo sapiens
gaatcttctggaagacctgg

SEQ ID NO: 1507 - DNA, 20 bp, homo sapiens
aatcttctggaagacctggc

SEQ ID NO: 1508 - DNA, 20 bp, homo sapiens
atcttctggaagacctggcg

SEQ ID NO: 1509 - DNA, 20 bp, homo sapiens
cgggtagtagcggccccgcc

SEQ ID NO: 1510 - DNA, 20 bp, homo sapiens
gggccgctactacccgctgc

SEQ ID NO: 1511 - DNA, 20 bp, homo sapiens
tggcctgcagcgggtagtag

SEQ ID NO: 1512 - DNA, 20 bp, homo sapiens
acatggtggtggcctgcagc

SEQ ID NO: 1513 - DNA, 20 bp, homo sapiens
aacatggtggtggcctgcag

SEQ ID NO: 1514 - DNA, 20 bp, homo sapiens
gggctggatcaacatggtgg

SEQ ID NO: 1515 - DNA, 20 bp, homo sapiens
catgggctggatcaacatgg

SEQ ID NO: 1516 - DNA, 20 bp, homo sapiens
caccatgttgatccagccca

SEQ ID NO: 1517 - DNA, 20 bp, homo sapiens
tgccatgggctggatcaaca

SEQ ID NO: 1518 - DNA, 20 bp, homo sapiens
gatccagcccatggcagcag

SEQ ID NO: 1519 - DNA, 20 bp, homo sapiens
ctgcctctgctgccatgggc

SEQ ID NO: 1520 - DNA, 20 bp, homo sapiens
gaggctgcctctgctgccat

SEQ ID NO: 1521 - DNA, 20 bp, homo sapiens
ggaggctgcctctgctgcca

SEQ ID NO: 1522 - DNA, 20 bp, homo sapiens
ggcccagccaggacgctagg